European Patent Application EP 4 575 505 A2, published June 25, 2025. Title: BIOMARKERS AND METHODS FOR PREDICTING PRETERM BIRTH. Applicant: SERA PROGNOSTICS, INC. Application EP. The sequence listing filed with the application follows.

SEQUENCE LISTING (1069 sequences)

SEQ ID NO: 1 - protein, 13 aa, Homo sapiens
AFTECCVVASQLR

SEQ ID NO: 2 - protein, 10 aa, Homo sapiens
ELLESYIDGR

SEQ ID NO: 3 - protein, 11 aa, Homo sapiens
ITLPDFTGDLR

SEQ ID NO: 4 - protein, 6 aa, Homo sapiens
FLNWIK

SEQ ID NO: 5 - protein, 13 aa, Homo sapiens
FGFGGSTDSGPIR

SEQ ID NO: 6 - protein, 8 aa, Homo sapiens
LLELTGPK

SEQ ID NO: 7 - protein, 10 aa, Homo sapiens
VEHSDLSFSK

SEQ ID NO: 8 - protein, 15 aa, Homo sapiens
IEGNLIFDPNNYLPK

SEQ ID NO: 9 - protein, 8 aa, Homo sapiens
ALVLELAK

SEQ ID NO: 10 - protein, 10 aa, Homo sapiens
TQILEWAAER

SEQ ID NO: 11 - protein, 20 aa, Homo sapiens
DVLLLVHNLPQNLPGYFWYK

SEQ ID NO: 12 - protein, 10 aa, Homo sapiens
SEPRPGVLLR

SEQ ID NO: 13 - protein, 8 aa, Homo sapiens
ITQDAQLK

SEQ ID NO: 14 - protein, 7 aa, Homo sapiens
ALDLSLK

SEQ ID NO: 15 - protein, 13 aa, Homo sapiens
WWGGQPLWITATK

SEQ ID NO: 16 - protein, 6 aa, Homo sapiens
LSETNR

SEQ ID NO: 17 - protein, 13 aa, Homo sapiens
TDAPDLPEENQAR

SEQ ID NO: 18 - protein, 8 aa, Homo sapiens
SFRPFVPR

SEQ ID NO: 19 - protein, 14 aa, Homo sapiens
LEQGENVFLQATDK

SEQ ID NO: 20 - protein, 12 aa, Homo sapiens
ETAASLLQAGYK

SEQ ID NO: 21 - protein, 8 aa, Homo sapiens
VTGWGNLK

SEQ ID NO: 22 - protein, 10 aa, Homo sapiens
EAQLPVIENK

SEQ ID NO: 23 - protein, 8 aa, Homo sapiens
FLQEQGHR

SEQ ID NO: 24 - protein, 8 aa, Homo sapiens
IRPFFPQQ

SEQ ID NO: 25 - protein, 11 aa, Homo sapiens
TLLPVSKPEIR

SEQ ID NO: 26 - protein, 10 aa, Homo sapiens
LSSPAVITDK

SEQ ID NO: 27 - protein, 15 aa, Homo sapiens
YEVQGEVFTKPQLWP

SEQ ID NO: 28 - protein, 10 aa, Homo sapiens
LQGTLPVEAR

SEQ ID NO: 29 - protein, 8 aa, Homo sapiens
VRPQQLVK

SEQ ID NO: 30 - protein, 7 aa, Homo sapiens
IEEIAAK

SEQ ID NO: 31 - protein, 16 aa, Homo sapiens
VQEAHLTEDQIFYFPK

SEQ ID NO: 32 - protein, 14 aa, Homo sapiens
ISLLLIESWLEPVR

SEQ ID NO: 33 - protein, 12 aa, Homo sapiens
ALQDQLVLVAAK

SEQ ID NO: 34 - protein, 7 aa, Homo sapiens
YEFLNGR

SEQ ID NO: 35 - protein, 18 aa, Homo sapiens
TPSAAYLWVGTGASEAEK

SEQ ID NO: 36 - protein, 13 aa, Homo sapiens
TATSEYQTFFNPR

SEQ ID NO: 37 - protein, 8 aa, Homo sapiens
TASDFITK

SEQ ID NO: 38 - protein, 18 aa, Homo sapiens
IITGLLEFEVYLEYLQNR

SEQ ID NO: 39 - protein, 10 aa, Homo sapiens
IIGGSDADIK

SEQ ID NO: 40 - protein, 7 aa, Homo sapiens
YTTEIIK

SEQ ID NO: 41 - protein, 12 aa, Homo sapiens
EDTPNSVWEPAK

SEQ ID NO: 42 - protein, 8 aa, Homo sapiens
LYYGDDEK

SEQ ID NO: 43 - protein, 8 aa, Homo sapiens
GGEIEGFR

SEQ ID NO: 44 - protein, 20 aa, Homo sapiens
DGSPDVTTADIGANTPDATK

SEQ ID NO: 45 - protein, 6 aa, Homo sapiens
VEIDTK

SEQ ID NO: 46 - protein, 8 aa, Homo sapiens
AVLTIDEK

SEQ ID NO: 47 - protein, 7 aa, Homo sapiens
FSVVYAK

SEQ ID NO: 48 - protein, 7 aa, Homo sapiens
YYLQGAK

SEQ ID NO: 49 - protein, 13 aa, Homo sapiens
EENFYVDETTVVK

SEQ ID NO: 50 - protein, 9 aa, Homo sapiens
YGFYTHVFR

SEQ ID NO: 51 - protein, 10 aa, Homo sapiens
HTLNQIDEVK

SEQ ID NO: 52 - protein, 12 aa, Homo sapiens
AFIQLWAFDAVK

SEQ ID NO: 53 - protein, 8 aa, Homo sapiens
SGFSFGFK

SEQ ID NO: 54 - protein, 11 aa, Homo sapiens
GWVTDGFSSLK

SEQ ID NO: 55 - protein, 14 aa, Homo sapiens
ITENDIQIALDDAK

SEQ ID NO: 56 - protein, 20 aa, Homo sapiens
VEPLYELVTATDFAYSSTVR

SEQ ID NO: 57 - protein, 22 aa, Homo sapiens
DPDQTDGLGLSYLSSHIANVER

SEQ ID NO: 58 - protein, 10 aa, Homo sapiens
VGEYSLYIGR

SEQ ID NO: 59 - protein, 15 aa, Homo sapiens
SLPVSDSVLSGFEQR

SEQ ID NO: 60 - protein, 10 aa, Homo sapiens
NADYSYSVWK

SEQ ID NO: 61 - protein, 10 aa, Homo sapiens
DAQYAPGYDK

SEQ ID NO: 62 - protein, 7 aa, Homo sapiens
FQLPGQK

SEQ ID NO: 63 - protein, 11 aa, Homo sapiens
YGLVTYATYPK

SEQ ID NO: 64 - protein, 18 aa, Homo sapiens
GSFALSFPVESDVAPIAR

SEQ ID NO: 65 - protein, 10 aa, Homo sapiens
TLLIANETLR

SEQ ID NO: 66 - protein, 22 aa, Homo sapiens
VILGAHQEVNLEPHVQEIEVSR

SEQ ID NO: 67 - protein, 9 aa, Homo sapiens
DISEVVTPR

SEQ ID NO: 68 - protein, 9 aa, Homo sapiens
TLEAQLTPR

SEQ ID NO: 69 - protein, 11 aa, Homo sapiens
AVGYLITGYQR

SEQ ID NO: 70 - protein, 18 aa, Homo sapiens
FNAVLTNPQGDYDTSTGK

SEQ ID NO: 71 - protein, 16 aa, Homo sapiens
SPEQQETVLDGNLIIR

SEQ ID NO: 72 - protein, 16 aa, Homo sapiens
ALNHLPLEYNSALYSR

SEQ ID NO: 73 - protein, 14 aa, Homo sapiens
GGEGTGYFVDFSVR

SEQ ID NO: 74 - protein, 9 aa, Homo sapiens
GIVEECCFR

SEQ ID NO: 75 - protein, 7 aa, Homo sapiens
FAFNLYR

SEQ ID NO: 76 - protein, 23 aa, Homo sapiens
AITPPHPASQANIIFDITEGNLR

SEQ ID NO: 77 - protein, 11 aa, Homo sapiens
EPGLCTWQSLR

SEQ ID NO: 78 - protein, 8 aa, Homo sapiens
AVYEAVLR

SEQ ID NO: 79 - protein, 6 aa, Homo sapiens
AWVAWR

SEQ ID NO: 80 - protein, 11 aa, Homo sapiens
TNLESILSYPK

SEQ ID NO: 81 - protein, 11 aa, Homo sapiens
HLSLLTTLSNR

SEQ ID NO: 82 - protein, 22 aa, Homo sapiens
FTFTLHLETPKPSISSSNLNPR

SEQ ID NO: 83 - protein, 16 aa, Homo sapiens
TELRPGETLNVNFLLR

SEQ ID NO: 84 - protein, 9 aa, Homo sapiens
LPTAVVPLR

SEQ ID NO: 85 - protein, 8 aa, Homo sapiens
APLTKPLK

SEQ ID NO: 86 - protein, 24 aa, Homo sapiens
ADSQAQLLLSTVVGVFTAPGLHLK

SEQ ID NO: 87 - protein, 8 aa, Homo sapiens
ELPEHTVK

SEQ ID NO: 88 - protein, 6 aa, Homo sapiens
AHYDLR

SEQ ID NO: 89 - protein, 13 aa, Homo sapiens
AEAQAQYSAAVAK

SEQ ID NO: 90 - protein, 7 aa, Homo sapiens
AYSDLSR

SEQ ID NO: 91 - protein, 16 aa, Homo sapiens
DALSSVQESQVAQQAR

SEQ ID NO: 92 - protein, 10 aa, Homo sapiens
ANRPFLVFIR

SEQ ID NO: 93 - protein, 11 aa, Homo sapiens
ALEQDLPVNIK

SEQ ID NO: 94 - protein, 14 aa, Homo sapiens
DFHINLFQVLPWLK

SEQ ID NO: 95 - protein, 14 aa, Homo sapiens
AGLLRPDYALLGHR

SEQ ID NO: 96 - protein, 19 aa, Homo sapiens
EKPAGGIPVLGSLVNTVLK

SEQ ID NO: 97 - protein, 9 aa, Homo sapiens
ITGFLKPGK

SEQ ID NO: 98 - protein, 7 aa, Homo sapiens
SLLQPNK

SEQ ID NO: 99 - protein, 9 aa, Homo sapiens
SPELQAEAK

SEQ ID NO: 100 - protein, 10 aa, Homo sapiens
TYLHTYESEI

SEQ ID NO: 101 - protein, 12 aa, Homo sapiens
DSPSVWAAVPGK

SEQ ID NO: 102 - protein, 8 aa, Homo sapiens
HYINLITR

SEQ ID NO: 103 - protein, 15 aa, Homo sapiens
IPGIFELGISSQSDR

SEQ ID NO: 104 - protein, 9 aa, Homo sapiens
IQTHSTTYR

SEQ ID NO: 105 - protein, 19 aa, Homo sapiens
QLGLPGPPDVPDHAAYHPF

SEQ ID NO: 106 - protein, 22 aa, Homo sapiens
FPLGSYTIQNIVAGSTYLFSTK

SEQ ID NO: 107 - protein, 13 aa, Homo sapiens
KLVIFDTMLEIKK

SEQ ID NO: 108 - protein, 30 aa, Homo sapiens
KFIEDNIEYITIIAFAQYVQEATFEEMEKL

SEQ ID NO: 109 - protein, 18 aa, Homo sapiens
KIAPQLSTEELVSLGEKM

SEQ ID NO: 110 - protein, 25 aa, Homo sapiens
KLKHELTDEELQSLFTNFANVVDKC

SEQ ID NO: 111 - protein, 11 aa, Homo sapiens
KLPNNVLQEKI

SEQ ID NO: 112 - protein, 19 aa, Homo sapiens
KSDVGFLPPFPTLDPEEKC

SEQ ID NO: 113 - protein, 10 aa, Homo sapiens
KVMNHICSKQ

SEQ ID NO: 114 - protein, 15 aa, Homo sapiens
RESLLNHFLYEVARR

SEQ ID NO: 115 - protein, 10 aa, Homo sapiens
RLCFFYNKKS

SEQ ID NO: 116 - protein, 21 aa, Homo sapiens
KAVLDVFEEGTEASAATAVKI

SEQ ID NO: 117 - protein, 10 aa, Homo sapiens
KEQLSLLDRF

SEQ ID NO: 118 - protein, 16 aa, Homo sapiens
KEQLSLLDRFTEDAKR

SEQ ID NO: 119 - protein, 17 aa, Homo sapiens
KEQLSLLDRFTEDAKRL

SEQ ID NO: 120 - protein, 25 aa, Homo sapiens
KITDLIKDLDSQTMMVLVNYIFFKA

SEQ ID NO: 121 - protein, 13 aa, Homo sapiens
KITLLSALVETRT

SEQ ID NO: 122 - protein, 21 aa, Homo sapiens
KRLYGSEAFATDFQDSAAAKK

SEQ ID NO: 123 - protein, 11 aa, Homo sapiens
REIGELYLPKF

SEQ ID NO: 124 - protein, 16 aa, Homo sapiens
RCEGPIPDVTFELLRE

SEQ ID NO: 125 - protein, 7 aa, Homo sapiens
RFALVRE

SEQ ID NO: 126 - protein, 10 aa, Homo sapiens
KSPPGVCSRD

SEQ ID NO: 127 - protein, 21 aa, Homo sapiens
RDSFHLDEQFTVPVEMMQART

SEQ ID NO: 128 - protein, 9 aa, Homo sapiens
KCNLLAEKQ

SEQ ID NO: 129 - protein, 16 aa, Homo sapiens
KEHAVEGDCDFQLLKL

SEQ ID NO: 130 - protein, 44 aa, Homo sapiens
KHTLNQIDEVKVWPQQPSGELFEIEIDTLETTCHVLDPTPVARC

SEQ ID NO: 131 - protein, 15 aa, Homo sapiens
KMVSGFIPLKPTVKM

SEQ ID NO: 132 - protein, 19 aa, Homo sapiens
RAFQPFFVELTMPYSVIRG

SEQ ID NO: 133 - protein, 15 aa, Homo sapiens
RNQGNTWLTAFVLKT

SEQ ID NO: 134 - protein, 14 aa, Homo sapiens
KIDRFMQAVTGWKT

SEQ ID NO: 135 - protein, 10 aa, Homo sapiens
KLDTEDKLRA

SEQ ID NO: 136 - protein, 27 aa, Homo sapiens
KTGCSLMGASVDSTLAFNTYVHFQGKM

SEQ ID NO: 137 - protein, 16 aa, Homo sapiens
RAAMVGMLANFLGFRI

SEQ ID NO: 138 - protein, 23 aa, Homo sapiens
KNDNDNIFLSPLSISTAFAMTKL

SEQ ID NO: 139 - protein, 24 aa, Homo sapiens
KSKLPGIVAEGRDDLYVSDAFHKA

SEQ ID NO: 140 - protein, 14 aa, Homo sapiens
REVPLNTIIFMGRV

SEQ ID NO: 141 - protein, 36 aa, Homo sapiens
RFATTFYQHLADSKNDNDNIFLSPLSISTAFAMTKL

SEQ ID NO: 142 - protein, 27 aa, Homo sapiens
RITDVIPSEAINELTVLVLVNTIYFKG

SEQ ID NO: 143 - protein, 9 aa, Homo sapiens
RRVWELSKA

SEQ ID NO: 144 - protein, 30 aa, Homo sapiens
RVAEGTQVLELPFKGDDITMVLILPKPEKS

SEQ ID NO: 145 - protein, 23 aa, Homo sapiens
KAGTELVNFLSYFVELGTQPATQ

SEQ ID NO: 146 - protein, 22 aa, Homo sapiens
KEPCVESLVSQYFQTVTDYGKD

SEQ ID NO: 147 - protein, 12 aa, Homo sapiens
KALVQQMEQLRQ

SEQ ID NO: 148 - protein, 19 aa, Homo sapiens
KLGPHAGDVEGHLSFLEKD

SEQ ID NO: 149 - protein, 16 aa, Homo sapiens
KSELTQQLNALFQDKL

SEQ ID NO: 150 - protein, 20 aa, Homo sapiens
KSLAELGGHLDQQVEEFRRR

SEQ ID NO: 151 - protein, 14 aa, Homo sapiens
KVKIDQTVEELRRS

SEQ ID NO: 152 - protein, 11 aa, Homo sapiens
KVNSFFSTFKE

SEQ ID NO: 153 - protein, 18 aa, Homo sapiens
KATFQTPDFIVPLTDLRI

SEQ ID NO: 154 - protein, 17 aa, Homo sapiens
KAVSMPSFSILGSDVRV

SEQ ID NO: 155 - protein, 13 aa, Homo sapiens
KEQHLFLPFSYKN

SEQ ID NO: 156 - protein, 13 aa, Homo sapiens
KKIISDYHQQFRY

SEQ ID NO: 157 - protein, 20 aa, Homo sapiens
KQVFLYPEKDEPTYILNIKR

SEQ ID NO: 158 - protein, 12 aa, Homo sapiens
KSPAFTDLHLRY

SEQ ID NO: 159 - protein, 20 aa, Homo sapiens
KTILGTMPAFEVSLQALQKA

SEQ ID NO: 160 - protein, 14 aa, Homo sapiens
KVLADKFIIPGLKL

SEQ ID NO: 161 - protein, 32 aa, Homo sapiens
KYSQPEDSLIPFFEITVPESQLTVSQFTLPKS

SEQ ID NO: 162 - protein, 13 aa, Homo sapiens
RDLKVEDIPLARI

SEQ ID NO: 163 - protein, 18 aa, Homo sapiens
RGIISALLVPPETEEAKQ

SEQ ID NO: 164 - protein, 21 aa, Homo sapiens
RILGEELGFASLHDLQLLGKL

SEQ ID NO: 165 - protein, 26 aa, Homo sapiens
RLELELRPTGEIEQYSVSATYELQRE

SEQ ID NO: 166 - protein, 17 aa, Homo sapiens
RNIQEYLSILTDPDGKG

SEQ ID NO: 167 - protein, 34 aa, Homo sapiens
RTFQIPGYTVPVVNVEVSPFTIEMSAFGYVFPKA

SEQ ID NO: 168 - protein, 22 aa, Homo sapiens
RTIDQMLNSELQWPVPDIYLRD

SEQ ID NO: 169 - protein, 13 aa, Homo sapiens
KMREWFSETFQKV

SEQ ID NO: 170 - protein, 25 aa, Homo sapiens
KSTAAMSTYTGIFTDQVLSVLKGEE

SEQ ID NO: 171 - protein, 13 aa, Homo sapiens
RGWVTDGFSSLKD

SEQ ID NO: 172 - protein, 17 aa, Homo sapiens
RAATVGSLAGQPLQERA

SEQ ID NO: 173 - protein, 16 aa, Homo sapiens
RLKSWFEPLVEDMQRQ

SEQ ID NO: 174 - protein, 25 aa, Homo sapiens
RWVQTLSEQVQEELLSSQVTQELRA

SEQ ID NO: 175 - protein, 13 aa, Homo sapiens
KLCGGGRWELMRI

SEQ ID NO: 176 - protein, 8 aa, Homo sapiens
KLPGLLKR

SEQ ID NO: 177 - protein, 11 aa, Homo sapiens
KEHSSLAFWKT

SEQ ID NO: 178 - protein, 19 aa, Homo sapiens
RTCPKPDDLPFSTVVPLKT

SEQ ID NO: 179 - protein, 16 aa, Homo sapiens
RVCPFAGILENGAVRY

SEQ ID NO: 180 - protein, 14 aa, Homo sapiens
KLFAAFFLEMAQLH

SEQ ID NO: 181 - protein, 12 aa, Homo sapiens
KSHLIIAQVAKN

SEQ ID NO: 182 - protein, 14 aa, Homo sapiens
KNAIWIDCGIHARE

SEQ ID NO: 183 - protein, 17 aa, Homo sapiens
REALIQFLEQVHQGIKG

SEQ ID NO: 184 - protein, 17 aa, Homo sapiens
RLLNIQTYCAGPAYLKG

SEQ ID NO: 185 - protein, 20 aa, Homo sapiens
RLCENIAGHLKDAQIFIQKK

SEQ ID NO: 186 - protein, 14 aa, Homo sapiens
KAETGDKVYVHLKN

SEQ ID NO: 187 - protein, 16 aa, Homo sapiens
KAGLQAFFQVQECNKS

SEQ ID NO: 188 - protein, 16 aa, Homo sapiens
KDIASGLIGPLIICKK

SEQ ID NO: 189 - protein, 13 aa, Homo sapiens
KDIFTGLIGPMKI

SEQ ID NO: 190 - protein, 23 aa, Homo sapiens
KMYYSAVDPTKDIFTGLIGPMKI

SEQ ID NO: 191 - protein, 14 aa, Homo sapiens
KPVWLGFLGPIIKA

SEQ ID NO: 192 - protein, 35 aa, Homo sapiens
RADDKVYPGEQYTYMLLATEEQSPGEGDGNCVTRI

SEQ ID NO: 193 - protein, 40 aa, Homo sapiens
RDTANLFPQTSLTLHMWPDTEGTFNVECLTTDHYTGGMKQ

SEQ ID NO: 194 - protein, 21 aa, Homo sapiens
RFNKNNEGTYYSPNYNPQSRS

SEQ ID NO: 195 - protein, 37 aa, Homo sapiens
RIDTINLFPATLFDAYMVAQNPGEWMLSCQNLNHLKA

SEQ ID NO: 196 - protein, 25 aa, Homo sapiens
RKAEEEHLGILGPQLHADVGDKVKI

SEQ ID NO: 197 - protein, 19 aa, Homo sapiens
RTTIEKPVWLGFLGPIIKA

SEQ ID NO: 198 - protein, 10 aa, Homo sapiens
RFWTSFFPKV

SEQ ID NO: 199 - protein, 19 aa, Homo sapiens
KLFDSDPITVTVPVEVSRK

SEQ ID NO: 200 - protein, 14 aa, Homo sapiens
RASSIIDELFQDRF

SEQ ID NO: 201 - protein, 16 aa, Homo sapiens
KWIVTAAHCVETGVKI

SEQ ID NO: 202 - protein, 15 aa, Homo sapiens
RFSLVSGWGQLLDRG

SEQ ID NO: 203 - protein, 13 aa, Homo sapiens
KETYDFDIAVLRL

SEQ ID NO: 204 - protein, 19 aa, Homo sapiens
KVRQLEMEIGQLNVHYLRN

SEQ ID NO: 205 - protein, 9 aa, Homo sapiens
RPAFSAIRR

SEQ ID NO: 206 - protein, 24 aa, Homo sapiens
KVVTFCDYAYNTFQVTTGGMVLKL

SEQ ID NO: 207 - protein, 11 aa, Homo sapiens
KFQSVFTVTRQ

SEQ ID NO: 208 - protein, 20 aa, Homo sapiens
KTLDEFTIIQNLQPQYQFRD

SEQ ID NO: 209 - protein, 19 aa, Homo sapiens
RMDVFSQNMFCAGHPSLKQ

SEQ ID NO: 210 - protein, 14 aa, Homo sapiens
RWILTAAHTLYPKE

SEQ ID NO: 211 - protein, 23 aa, Homo sapiens
KFYAAGLVSWGPQCGTYGLYTRV

SEQ ID NO: 212 - protein, 11 aa, Homo sapiens
KGFQVVVTLRR

SEQ ID NO: 213 - protein, 19 aa, Homo sapiens
RGALISDQWVLTAAHCFRD

SEQ ID NO: 214 - protein, 17 aa, Homo sapiens
RPICLPCTMEANLALRR

SEQ ID NO: 215 - protein, 26 aa, Homo sapiens
RYYGGGYGSTQATFMVFQALAQYQKD

SEQ ID NO: 216 - protein, 13 aa, Homo sapiens
KGLCVATPVQLRV

SEQ ID NO: 217 - protein, 21 aa, Homo sapiens
KMRPSTDTITVMVENSHGLRV

SEQ ID NO: 218 - protein, 23 aa, Homo sapiens
KVGLSGMAIADVTLLSGFHALRA

SEQ ID NO: 219 - protein, 17 aa, Homo sapiens
KVLSLAQEQVGGSPEKL

SEQ ID NO: 220 - protein, 15 aa, Homo sapiens
REMSGSPASGIPVKV

SEQ ID NO: 221 - protein, 20 aa, Homo sapiens
RGCGEQTMIYLAPTLAASRY

SEQ ID NO: 222 - protein, 11 aa, Homo sapiens
RGLQDEDGYRM

SEQ ID NO: 223 - protein, 13 aa, Homo sapiens
RGQIVFMNREPKR

SEQ ID NO: 224 - protein, 29 aa, Homo sapiens
RKKEVYMPSSIFQDDFVIPDISEPGTWKI

SEQ ID NO: 225 - protein, 8 aa, Homo sapiens
RLPMSVRR

SEQ ID NO: 226 - protein, 20 aa, Homo sapiens
RLTVAAPPSGGPGFLSIERP

SEQ ID NO: 227 - protein, 7 aa, Homo sapiens
RNFLVRA

SEQ ID NO: 228 - protein, 34 aa, Homo sapiens
RNGESVKLHLETDSLALVALGALDTALYAAGSKS

SEQ ID NO: 229 - protein, 11 aa, Homo sapiens
RQGSFQGGFRS

SEQ ID NO: 230 - protein, 25 aa, Homo sapiens
RTLEIPGNSDPNMIPDGDFNSYVRV

SEQ ID NO: 231 - protein, 28 aa, Homo sapiens
RVTASDPLDTLGSEGALSPGGVASLLRL

SEQ ID NO: 232 - protein, 18 aa, Homo sapiens
RYLDKTEQWSTLPPETKD

SEQ ID NO: 233 - protein, 32 aa, Homo sapiens
KADNFLLENTLPAQSTFTLAISAYALSLGDKT

SEQ ID NO: 234 - protein, 18 aa, Homo sapiens
KALVEGVDQLFTDYQIKD

SEQ ID NO: 235 - protein, 22 aa, Homo sapiens
KDGHVILQLNSIPSSDFLCVRF

SEQ ID NO: 236 - protein, 16 aa, Homo sapiens
KDVFLEMNIPYSVVRG

SEQ ID NO: 237 - protein, 15 aa, Homo sapiens
KEFPYRIPLDLVPKT

SEQ ID NO: 238 - protein, 14 aa, Homo sapiens
KFQNSAILTIQPKQ

SEQ ID NO: 239 - protein, 19 aa, Homo sapiens
KVFKDVFLEMNIPYSVVRG

SEQ ID NO: 240 - protein, 9 aa, Homo sapiens
RVFQFLEKS

SEQ ID NO: 241 - protein, 12 aa, Homo sapiens
KDLHLSDVFLKA

SEQ ID NO: 242 - protein, 21 aa, Homo sapiens
RTECIKPVVQEVLTITPFQRL

SEQ ID NO: 243 - protein, 11 aa, Homo sapiens
KSSGWHFVVKF

SEQ ID NO: 244 - protein, 10 aa, Homo sapiens
RILPLTVCKM

SEQ ID NO: 245 - protein, 15 aa, Homo sapiens
RALDQYLMEFNACRC

SEQ ID NO: 246 - protein, 19 aa, Homo sapiens
KYGFCEAADQFHVLDEVRR

SEQ ID NO: 247 - protein, 15 aa, Homo sapiens
RAIEDYINEFSVRKC

SEQ ID NO: 248 - protein, 31 aa, Homo sapiens
RTAGYGINILGMDPLSTPFDNEFYNGLCNRD

SEQ ID NO: 249 - protein, 12 aa, Homo sapiens
KALFVSEEEKKL

SEQ ID NO: 250 - protein, 10 aa, Homo sapiens
KCLVNLIEKV

SEQ ID NO: 251 - protein, 18 aa, Homo sapiens
KEAGIPEFYDYDVALIKL

SEQ ID NO: 252 - protein, 16 aa, Homo sapiens
KVSEADSSNADWVTKQ

SEQ ID NO: 253 - protein, 20 aa, Homo sapiens
KYGQTIRPICLPCTEGTTRA

SEQ ID NO: 254 - protein, 20 aa, Homo sapiens
RDLEIEVVLFHPNYNINGKK

SEQ ID NO: 255 - protein, 19 aa, Homo sapiens
RFLCTGGVSPYADPNTCRG

SEQ ID NO: 256 - protein, 13 aa, Homo sapiens
KDGWSAQPTCIKS

SEQ ID NO: 257 - protein, 14 aa, Homo sapiens
KEGWIHTVCINGRW

SEQ ID NO: 258 - protein, 20 aa, Homo sapiens
KTDCLSLPSFENAIPMGEKK

SEQ ID NO: 259 - protein, 20 aa, Homo sapiens
RDTSCVNPPTVQNAYIVSRQ

SEQ ID NO: 260 - protein, 13 aa, Homo sapiens
KCTSTGWIPAPRC

SEQ ID NO: 261 - protein, 10 aa, Homo sapiens
KIIYKENERF

SEQ ID NO: 262 - protein, 21 aa, Homo sapiens
KIVSSAMEPDREYHFGQAVRF

SEQ ID NO: 263 - protein, 14 aa, Homo sapiens
RCTLKPCDYPDIKH

SEQ ID NO: 264 - protein, 13 aa, Homo sapiens
RKGEWVALNPLRK

SEQ ID NO: 265 - protein, 14 aa, Homo sapiens
RKGEWVALNPLRKC

SEQ ID NO: 266 - protein, 12 aa, Homo sapiens
RRPYFPVAVGKY

SEQ ID NO: 267 - protein, 13 aa, Homo sapiens
REIMENYNIALRW

SEQ ID NO: 268 - protein, 27 aa, Homo sapiens
KDASGITCGGIYIGGCWILTAAHCLRA

SEQ ID NO: 269 - protein, 16 aa, Homo sapiens
KVANYFDWISYHVGRP

SEQ ID NO: 270 - protein, 24 aa, Homo sapiens
RIIFHENYNAGTYQNDIALIEMKK

SEQ ID NO: 271 - protein, 18 aa, Homo sapiens
RYQIWTTVVDWIHPDLKR

SEQ ID NO: 272 - protein, 8 aa, Homo sapiens
KISNLLKF

SEQ ID NO: 273 - protein, 18 aa, Homo sapiens
RWSAGLTSSQVDLYIPKV

SEQ ID NO: 274 - protein, 16 aa, Homo sapiens
KYEVQGEVFTKPQLWP

SEQ ID NO: 275 - protein, 13 aa, Homo sapiens
RHVLAAWALGAKA

SEQ ID NO: 276 - protein, 16 aa, Homo sapiens
RAGLRYVCLAEPAERR

SEQ ID NO: 277 - protein, 19 aa, Homo sapiens
RFTQLCVKGGGGGGNGIRD

SEQ ID NO: 278 - protein, 19 aa, Homo sapiens
RVQLGPYQPGRPAACDLRE

SEQ ID NO: 279 - protein, 24 aa, Homo sapiens
RGGLGSLFYLTLDVLETDCHVLRK

SEQ ID NO: 280 - protein, 23 aa, Homo sapiens
RELLSQGATLSGWYHLCLPEGRA

SEQ ID NO: 281 - protein, 16 aa, Homo sapiens
KKTTDMILNEIKQGKF

SEQ ID NO: 282 - protein, 27 aa, Homo sapiens
KNWRDPDQTDGLGLSYLSSHIANVERV

SEQ ID NO: 283 - protein, 20 aa, Homo sapiens
KTPSAAYLWVGTGASEAEKT

SEQ ID NO: 284 - protein, 29 aa, Homo sapiens
RVEKFDLVPVPTNLYGDFFTGDAYVILKT

SEQ ID NO: 285 - protein, 30 aa, Homo sapiens
RVPFDAATLHTSTAMAAQHGMDDDGTGQKQ

SEQ ID NO: 286 - protein, 8 aa, Homo sapiens
KFYTFLKN

SEQ ID NO: 287 - protein, 14 aa, Homo sapiens
KGDKVWVYPPEKKE

SEQ ID NO: 288 - protein, 23 aa, Homo sapiens
KLLQDEFPGIPSPLDAAVECHRG

SEQ ID NO: 289 - protein, 18 aa, Homo sapiens
KSGAQATWTELPWPHEKV

SEQ ID NO: 290 - protein, 27 aa, Homo sapiens
KSGAQATWTELPWPHEKVDGALCMEKS

SEQ ID NO: 291 - protein, 11 aa, Homo sapiens
KVDGALCMEKS

SEQ ID NO: 292 - protein, 11 aa, Homo sapiens
RDYFMPCPGRG

SEQ ID NO: 293 - protein, 14 aa, Homo sapiens
REWFWDLATGTMKE

SEQ ID NO: 294 - protein, 12 aa, Homo sapiens
RQGHNSVFLIKG

SEQ ID NO: 295 - protein, 32 aa, Homo sapiens
KHQGTITVNEEGTQATTVTTVGFMPLSTQVRF

SEQ ID NO: 296 - protein, 13 aa, Homo sapiens
KYEITTIHNLFRK

SEQ ID NO: 297 - protein, 9 aa, Homo sapiens
RLNILNAKF

SEQ ID NO: 298 - protein, 9 aa, Homo sapiens
RNFGYTLRS

SEQ ID NO: 299 - protein, 21 aa, Homo sapiens
RVQLSPDLLATLPEPASPGRQ

SEQ ID NO: 300 - protein, 11 aa, Homo sapiens
RDGYLFQLLRI

SEQ ID NO: 301 - protein, 8 aa, Homo sapiens
KFLNWIKA

SEQ ID NO: 302 - protein, 15 aa, Homo sapiens
KLKPVDGHCALESKY

SEQ ID NO: 303 - protein, 12 aa, Homo sapiens
KRPGVYTQVTKF

SEQ ID NO: 304 - protein, 23 aa, Homo sapiens
KAGADTHGRLLQGNICNDAVTKA

SEQ ID NO: 305 - protein, 16 aa, Homo sapiens
KKIIEKMATFEIDEKR

SEQ ID NO: 306 - protein, 24 aa, Homo sapiens
RSFEGLGQLEVLTLDHNQLQEVKA

SEQ ID NO: 307 - protein, 11 aa, Homo sapiens
KELAAQTIKKS

SEQ ID NO: 308 - protein, 21 aa, Homo sapiens
KGSLVQASEANLQAAQDFVRG

SEQ ID NO: 309 - protein, 22 aa, Homo sapiens
KQLVHHFEIDVDIFEPQGISKL

SEQ ID NO: 310 - protein, 15 aa, Homo sapiens
KQYYEGSEIVVAGRI

SEQ ID NO: 311 - protein, 33 aa, Homo sapiens
REVAFDLEIPKTAFISDFAVTADGNAFIGDIKD

SEQ ID NO: 312 - protein, 30 aa, Homo sapiens
RGMADQDGLKPTIDKPSEDSPPLEMLGPRR

SEQ ID NO: 313 - protein, 41 aa, Homo sapiens
KFDPAKLDQIESVITATSANTQLVLETLAQMDDLQDFLSKD

SEQ ID NO: 314 - protein, 14 aa, Homo sapiens
KKFYNQVSTPLLRN

SEQ ID NO: 315 - protein, 18 aa, Homo sapiens
KNILFVIDVSGSMWGVKM

SEQ ID NO: 316 - protein, 10 aa, Homo sapiens
RKLGSYEHRI

SEQ ID NO: 317 - protein, 13 aa, Homo sapiens
RLSNENHGIAQRI

SEQ ID NO: 318 - protein, 11 aa, Homo sapiens
RMATTMIQSKV

SEQ ID NO: 319 - protein, 30 aa, Homo sapiens
RSILQMSLDHHIVTPLTSLVIENEAGDERM

SEQ ID NO: 320 - protein, 12 aa, Homo sapiens
RTEVNVLPGAKV

SEQ ID NO: 321 - protein, 10 aa, Homo sapiens
KNVVFVIDKS

SEQ ID NO: 322 - protein, 15 aa, Homo sapiens
KWKETLFSVMPGLKM

SEQ ID NO: 323 - protein, 11 aa, Homo sapiens
KYIFHNFMERL

SEQ ID NO: 324 - protein, 11 aa, Homo sapiens
RFAHTVVTSRV

SEQ ID NO: 325 - protein, 12 aa, Homo sapiens
RFKPTLSQQQKS

SEQ ID NO: 326 - protein, 46 aa, Homo sapiens
RIHEDSDSALQLQDFYQEVANPLLTAVTFEYPSNAVEEVTQNNFRL

SEQ ID NO: 327 - protein, 13 aa, Homo sapiens
RMNFRPGVLSSRQ

SEQ ID NO: 328 - protein, 13 aa, Homo sapiens
RNVHSAGAAGSRM

SEQ ID NO: 329 - protein, 12 aa, Homo sapiens
RNVHSGSTFFKY

SEQ ID NO: 330 - protein, 12 aa, Homo sapiens
RRLGVYELLLKV

SEQ ID NO: 331 - protein, 10 aa, Homo sapiens
KKLELHLPKF

SEQ ID NO: 332 - protein, 15 aa, Homo sapiens
REIEEVLTPEMLMRW

SEQ ID NO: 333 - protein, 15 aa, Homo sapiens
KAATGECTATVGKRS

SEQ ID NO: 334 - protein, 20 aa, Homo sapiens
KLGQSLDCNAEVYVVPWEKK

SEQ ID NO: 335 - protein, 17 aa, Homo sapiens
KYNSQNQSNNQFVLYRI

SEQ ID NO: 336 - protein, 11 aa, Homo sapiens
RQVVAGLNFRI

SEQ ID NO: 337 - protein, 12 aa, Homo sapiens
KDLLLPQPDLRY

SEQ ID NO: 338 - protein, 15 aa, Homo sapiens
RLHLEGNKLQVLGKD

SEQ ID NO: 339 - protein, 20 aa, Homo sapiens
RTLDLGENQLETLPPDLLRG

SEQ ID NO: 340 - protein, 21 aa, Homo sapiens
KGLQYAAQEGLLALQSELLRI

SEQ ID NO: 341 - protein, 13 aa, Homo sapiens
KLAEGFPLPLLKR

SEQ ID NO: 342 - protein, 16 aa, Homo sapiens
KSLEYLDLSFNQIARL

SEQ ID NO: 343 - protein, 13 aa, Homo sapiens
RLKEDAVSAAFKG

SEQ ID NO: 344 - protein, 21 aa, Homo sapiens
RIVFENPDPSDGFVLIPDLKW

SEQ ID NO: 345 - protein, 7 aa, Homo sapiens
RVYFFKG

SEQ ID NO: 346 - protein, 8 aa, Homo sapiens
KWFDYLRE

SEQ ID NO: 347 - protein, 20 aa, Homo sapiens
RLTVGAAQVPAQLLVGALRV

SEQ ID NO: 348 - protein, 18 aa, Homo sapiens
RVSFSSPLVAISGVALRS

SEQ ID NO: 349 - protein, 19 aa, Homo sapiens
KGIVAAFYSGPSLSDKEKL

SEQ ID NO: 350 - protein, 16 aa, Homo sapiens
RWYVPVKDLLGIYEKL

SEQ ID NO: 351 - protein, 14 aa, Homo sapiens
KLQSLFDSPDFSKI

SEQ ID NO: 352 - protein, 19 aa, Homo sapiens
RALYYDLISSPDIHGTYKE

SEQ ID NO: 353 - protein, 20 aa, Homo sapiens
RCLLFSFLPASSINDMEKRF

SEQ ID NO: 354 - protein, 12 aa, Homo sapiens
KFQPTLLTLPRI

SEQ ID NO: 355 - protein, 19 aa, Homo sapiens
KGVTSVSQIFHSPDLAIRD

SEQ ID NO: 356 - protein, 18 aa, Homo sapiens
KVIPACLPSPNYVVADRT

SEQ ID NO: 357 - protein, 12 aa, Homo sapiens
RFVTWIEGVMRN

SEQ ID NO: 358 - protein, 13 aa, Homo sapiens
RHSIFTPETNPRA

SEQ ID NO: 359 - protein, 17 aa, Homo sapiens
KGKEESLDSDLYAELRC

SEQ ID NO: 360 - protein, 17 aa, Homo sapiens
KMVLLEQLFLDHNALRG

SEQ ID NO: 361 - protein, 24 aa, Homo sapiens
RLVSLDSGLLNSLGALTELQFHRN

SEQ ID NO: 362 - protein, 14 aa, Homo sapiens
KALLAYAFSLLGKQ

SEQ ID NO: 363 - protein, 14 aa, Homo sapiens
KDLFHCVSFTLPRI

SEQ ID NO: 364 - protein, 14 aa, Homo sapiens
KMLQITNTGFEMKL

SEQ ID NO: 365 - protein, 16 aa, Homo sapiens
RNELIPLIYLENPRRN

SEQ ID NO: 366 - protein, 24 aa, Homo sapiens
RSYIFIDEAHITQSLTWLSQMQKD

SEQ ID NO: 367 - protein, 18 aa, Homo sapiens
RSDPVTLNLLHGPDLPRI

SEQ ID NO: 368 - protein, 11 aa, Homo sapiens
RTLFLFGVTKY

SEQ ID NO: 369 - protein, 11 aa, Homo sapiens
RILILPSVTRN

SEQ ID NO: 370 - protein, 13 aa, Homo sapiens
RSDPVTLNLLPKL

SEQ ID NO: 371 - protein, 8 aa, Homo sapiens
RVLQLEKQ

SEQ ID NO: 372 - protein, 21 aa, Homo sapiens
RVVAQGVGIPEDSIFTMADRG

SEQ ID NO: 373 - protein, 28 aa, Homo sapiens
RLTEREWADEWKHLDHALNCIMEMVEKT

SEQ ID NO: 374 - protein, 21 aa, Homo sapiens
RALCGGDGAAALREPGAGLRL

SEQ ID NO: 375 - protein, 24 aa, Homo sapiens
KALMDLLAGKGSQGSQAPQALDRT

SEQ ID NO: 376 - protein, 23 aa, Homo sapiens
KMGDHLALEDYLTTDLVETWLRN

SEQ ID NO: 377 - protein, 17 aa, Homo sapiens
KSPQELLCGASLISDRW

SEQ ID NO: 378 - protein, 21 aa, Homo sapiens
RLAVTTHGLPCLAWASAQAKA

SEQ ID NO: 379 - protein, 21 aa, Homo sapiens
RSEGSSVNLSPPLEQCVPDRG

SEQ ID NO: 380 - protein, 11 aa, Homo sapiens
RSGIECQLWRS

SEQ ID NO: 381 - protein, 15 aa, Homo sapiens
RTATSEYQTFFNPRT

SEQ ID NO: 382 - protein, 19 aa, Homo sapiens
RVTGWGNLKETWTANVGKG

SEQ ID NO: 383 - protein, 9 aa, Homo sapiens
RIHLMAGRV

SEQ ID NO: 384 - protein, 9 aa, Homo sapiens
RPAHPALRL

SEQ ID NO: 385 - protein, 8 aa, Homo sapiens
KISNIIKQ

SEQ ID NO: 386 - protein, 14 aa, Homo sapiens
KMKYWGVASFLQKG

SEQ ID NO: 387 - protein, 12 aa, Homo sapiens
RFSGTWYAMAKK

SEQ ID NO: 388 - protein, 20 aa, Homo sapiens
RLLNLDGTCADSYSFVFSRD

SEQ ID NO: 389 - protein, 27 aa, Homo sapiens
RLLNNWDVCADMVGTFTDTEDPAKFKM

SEQ ID NO: 390 - protein, 28 aa, Homo sapiens
RLFLGALPGEDSSTSFCLNGLWAQGQRL

SEQ ID NO: 391 - protein, 11 aa, Homo sapiens
KDDWFMLGLRD

SEQ ID NO: 392 - protein, 25 aa, Homo sapiens
RSCDVESNPGIFLPPGTQAEFNLRG

SEQ ID NO: 393 - protein, 27 aa, Homo sapiens
RTWDPEGVIFYGDTNPKDDWFMLGLRD

SEQ ID NO: 394 - protein, 26 aa, Homo sapiens
RKFCRDIQDPTQLAEMIFNLLLEEKR

SEQ ID NO: 395 - protein, 16 aa, Homo sapiens
RNELIRQEKLEQLARR

SEQ ID NO: 396 - protein, 8 aa, Homo sapiens
RKNLSERW

SEQ ID NO: 397 - protein, 12 aa, Homo sapiens
RKWYNLMIQNKD

SEQ ID NO: 398 - protein, 16 aa, Homo sapiens
KSRLDTLAQEVALLKE

SEQ ID NO: 399 - protein, 16 aa, Homo sapiens
KRLDVNAAGIWEPKKG

SEQ ID NO: 400 - protein, 9 aa, Homo sapiens
RSILFLGKV

SEQ ID NO: 401 - protein, 28 aa, Homo sapiens
RELISDLEHRLQGSVMELLQGVDGVIKR

SEQ ID NO: 402 - protein, 27 aa, Homo sapiens
KELSSFIDKGQELCADYSENTFTEYKK

SEQ ID NO: 403 - protein, 28 aa, Homo sapiens
KELSSFIDKGQELCADYSENTFTEYKKK

SEQ ID NO: 404 - protein, 24 aa, Homo sapiens
KEVVSLTEACCAEGADPDCYDTRT

SEQ ID NO: 405 - protein, 40 aa, Homo sapiens
KTAMDVFVCTYFMPAAQLPELPDVELPTNKDVCDPGNTKV

SEQ ID NO: 406 - protein, 13 aa, Homo sapiens
RRTHLPEVFLSKV

SEQ ID NO: 407 - protein, 13 aa, Homo sapiens
RVCSQYAAYGEKK

SEQ ID NO: 408 - protein, 20 aa, Homo sapiens
KLIRDVWGIEGPIDAAFTRI

SEQ ID NO: 409 - protein, 17 aa, Homo sapiens
RDVWGIEGPIDAAFTRI

SEQ ID NO: 410 - protein, 9 aa, Homo sapiens
RERVYFFKG

SEQ ID NO: 411 - protein, 14 aa, Homo sapiens
RFEDGVLDPDYPRN

SEQ ID NO: 412 - protein, 16 aa, Homo sapiens
RIYISGMAPRPSLAKK

SEQ ID NO: 413 - protein, 8 aa, Homo sapiens
KTRFLLRT

SEQ ID NO: 414 - protein, 23 aa, Homo sapiens
KHELTDEELQSLFTNFANVVDKC

SEQ ID NO: 415 - protein, 23 aa, Homo sapiens
RNPFVFAPTLLTVAVHFEEVAKS

SEQ ID NO: 416 - protein, 12 aa, Homo sapiens
KADLSGITGARN

SEQ ID NO: 417 - protein, 17 aa, Homo sapiens
KMEEVEAMLLPETLKRW

SEQ ID NO: 418 - protein, 16 aa, Homo sapiens
KWEMPFDPQDTHQSRF

SEQ ID NO: 419 - protein, 20 aa, Homo sapiens
RLYGSEAFATDFQDSAAAKK

SEQ ID NO: 420 - protein, 14 aa, Homo sapiens
KHQFLLTGDTQGRY

SEQ ID NO: 421 - protein, 18 aa, Homo sapiens
KNGVAQEPVHLDSPAIKH

SEQ ID NO: 422 - protein, 22 aa, Homo sapiens
KSLPAPWLSMAPVSWITPGLKT

SEQ ID NO: 423 - protein, 20 aa, Homo sapiens
KVTLTCVAPLSGVDFQLRRG

SEQ ID NO: 424 - protein, 11 aa, Homo sapiens
RCLAPLEGARF

SEQ ID NO: 425 - protein, 9 aa, Homo sapiens
RGVTFLLRR

SEQ ID NO: 426 - protein, 39 aa, Homo sapiens
RLHDNQNGWSGDSAPVELILSDETLPAPEFSPEPESGRA

SEQ ID NO: 427 - protein, 24 aa, Homo sapiens
RTPGAAANLELIFVGPQHAGNYRC

SEQ ID NO: 428 - protein, 26 aa, Homo sapiens
KHQMDLVATLSQLGLQELFQAPDLRG

SEQ ID NO: 429 - protein, 13 aa, Homo sapiens
RLCQDLGPGAFRL

SEQ ID NO: 430 - protein, 19 aa, Homo sapiens
RWFLLEQPEIQVAHFPFKN

SEQ ID NO: 431 - protein, 34 aa, Homo sapiens
KVWPQQPSGELFEIEIDTLETTCHVLDPTPVARC

SEQ ID NO: 432 - protein, 22 aa, Homo sapiens
RHTFMGVVSLGSPSGEVSHPRK

SEQ ID NO: 433 - protein, 31 aa, Homo sapiens
RQPNCDDPETEEAALVAIDYINQNLPWGYKH

SEQ ID NO: 434 - protein, 23 aa, Homo sapiens
RTVVQPSVGAAAGPVVPPCPGRI

SEQ ID NO: 435 - protein, 19 aa, Homo sapiens
KQPFVQGLALYTPVVLPRS

SEQ ID NO: 436 - protein, 13 aa, Homo sapiens
KLVPFATELHERL

SEQ ID NO: 437 - protein, 13 aa, Homo sapiens
RLLPHANEVSQKI

SEQ ID NO: 438 - protein, 27 aa, Homo sapiens
RSLAPYAQDTQEKLNHQLEGLTFQMKK

SEQ ID NO: 439 - protein, 11 aa, Homo sapiens
KFPEVDVLTKY

SEQ ID NO: 440 - protein, 11 aa, Homo sapiens
KHINIDQFVRK

SEQ ID NO: 441 - protein, 17 aa, Homo sapiens
KLLSGGNTLHLVSTTKT

SEQ ID NO: 442 - protein, 21 aa, Homo sapiens
KQVFLYPEKDEPTYILNIKRG

SEQ ID NO: 443 - protein, 10 aa, Homo sapiens
KSLHMYANRL

SEQ ID NO: 444 - protein, 19 aa, Homo sapiens
KSVSDGIAALDLNAVANKI

SEQ ID NO: 445 - protein, 30 aa, Homo sapiens
KSVSLPSLDPASAKIEGNLIFDPNNYLPKE

SEQ ID NO: 446 - protein, 13 aa, Homo sapiens
KTEVIPPLIENRQ

SEQ ID NO: 447 - protein, 12 aa, Homo sapiens
KVLVDHFGYTKD

SEQ ID NO: 448 - protein, 26 aa, Homo sapiens
RTSSFALNLPTLPEVKFPEVDVLTKY

SEQ ID NO: 449 - protein, 20 aa, Homo sapiens
RGWVTDGFSSLKDYWSTVKD

SEQ ID NO: 450 - protein, 17 aa, Homo sapiens
RGEVQAMLGQSTEELRV

SEQ ID NO: 451 - protein, 11 aa, Homo sapiens
RLAVYQAGARE

SEQ ID NO: 452 - protein, 11 aa, Homo sapiens
RLGPLVEQGRV

SEQ ID NO: 453 - protein, 12 aa, Homo sapiens
KLTLTPWVGLRK

SEQ ID NO: 454 - protein, 17 aa, Homo sapiens
KFICPLTGLWPINTLKC

SEQ ID NO: 455 - protein, 22 aa, Homo sapiens
KTFYEPGEEITYSCKPGYVSRG

SEQ ID NO: 456 - protein, 27 aa, Homo sapiens
KMVVSMTLGLHPWIANIDDTQYLAAKR

SEQ ID NO: 457 - protein, 19 aa, Homo sapiens
KVFQYIDLHQDEFVQTLKE

SEQ ID NO: 458 - protein, 19 aa, Homo sapiens
RTSIYPFLDFMPSPQVVRW

SEQ ID NO: 459 - protein, 17 aa, Homo sapiens
RELMLQLSEFLCEEFRN

SEQ ID NO: 460 - protein, 24 aa, Homo sapiens
KAEEEHLGILGPQLHADVGDKVKI

SEQ ID NO: 461 - protein, 14 aa, Homo sapiens
KALYLQYTDETFRT

SEQ ID NO: 462 - protein, 28 aa, Homo sapiens
KDVDKEFYLFPTVFDENESLLLEDNIRM

SEQ ID NO: 463 - protein, 22 aa, Homo sapiens
KHYYIGIIETTWDYASDHGEKK

SEQ ID NO: 464 - protein, 13 aa, Homo sapiens
REYTDASFTNRKE

SEQ ID NO: 465 - protein, 25 aa, Homo sapiens
RHYYIAAEEIIWNYAPSGIDIFTKE

SEQ ID NO: 466 - protein, 12 aa, Homo sapiens
RIYHSHIDAPKD

SEQ ID NO: 467 - protein, 30 aa, Homo sapiens
RQKDVDKEFYLFPTVFDENESLLLEDNIRM

SEQ ID NO: 468 - protein, 19 aa, Homo sapiens
RTYYIAAVEVEWDYSPQRE

SEQ ID NO: 469 - protein, 11 aa, Homo sapiens
RSALVLQYLRV

SEQ ID NO: 470 - protein, 14 aa, Homo sapiens
KEFNPLVIVGLSKD

SEQ ID NO: 471 - protein, 17 aa, Homo sapiens
RNPDNDIRPWCFVLNRD

SEQ ID NO: 472 - protein, 11 aa, Homo sapiens
RVVGGLVALRG

SEQ ID NO: 473 - protein, 25 aa, Homo sapiens
KNSLLGMEGANSIFSGFLLFPDMEA

SEQ ID NO: 474 - protein, 16 aa, Homo sapiens
KVPGLYYFTYHASSRG

SEQ ID NO: 475 - protein, 15 aa, Homo sapiens
RQTHQPPAPNSLIRF

SEQ ID NO: 476 - protein, 16 aa, Homo sapiens
RLPVANPQACENWLRG

SEQ ID NO: 477 - protein, 18 aa, Homo sapiens
KNQGILEFYGDDIALLKL

SEQ ID NO: 478 - protein, 16 aa, Homo sapiens
KRNDYLDIYAIGVGKL

SEQ ID NO: 479 - protein, 33 aa, Homo sapiens
RQPYSYDFPEDVAPALGTSFSHMLGATNPTQKT

SEQ ID NO: 480 - protein, 12 aa, Homo sapiens
RIHWESASLLRS

SEQ ID NO: 481 - protein, 9 aa, Homo sapiens
KFACYYPRV

SEQ ID NO: 482 - protein, 28 aa, Homo sapiens
KLHLETDSLALVALGALDTALYAAGSKS

SEQ ID NO: 483 - protein, 14 aa, Homo sapiens
KLVNGQSHISLSKA

SEQ ID NO: 484 - protein, 11 aa, Homo sapiens
KSCGLHQLLRG

SEQ ID NO: 485 - protein, 11 aa, Homo sapiens
KYVLPNFEVKI

SEQ ID NO: 486 - protein, 21 aa, Homo sapiens
RALEILQEEDLIDEDDIPVRS

SEQ ID NO: 487 - protein, 33 aa, Homo sapiens
RECVGFEAVQEVPVGLVQPASATLYDYYNPERR

SEQ ID NO: 488 - protein, 15 aa, Homo sapiens
REELVYELNPLDHRG

SEQ ID NO: 489 - protein, 27 aa, Homo sapiens
RSTQDTVIALDALSAYWIASHTTEERG

SEQ ID NO: 490 - protein, 12 aa, Homo sapiens
RVGDTLNLNLRA

SEQ ID NO: 491 - protein, 11 aa, Homo sapiens
RVHYTVCIWRN

SEQ ID NO: 492 - protein, 12 aa, Homo sapiens
KKYVLPNFEVKI

SEQ ID NO: 493 - protein, 26 aa, Homo sapiens
KVDFTLSSERDFALLSLQVPLKDAKS

SEQ ID NO: 494 - protein, 18 aa, Homo sapiens
RSYFPESWLWEVHLVPRR

SEQ ID NO: 495 - protein, 28 aa, Homo sapiens
RYGGGFYSTQDTINAIEGLTEYSLLVKQ

SEQ ID NO: 496 - protein, 12 aa, Homo sapiens
RHTSLGPLEAKR

SEQ ID NO: 497 - protein, 35 aa, Homo sapiens
KCQHEMDQYWGIGSLASGINLFTNSFEGPVLDHRY

SEQ ID NO: 498 - protein, 10 aa, Homo sapiens
KSGFSFGFKI

SEQ ID NO: 499 - protein, 14 aa, Homo sapiens
RDTMVEDLVVLVRG

SEQ ID NO: 500 - protein, 24 aa, Homo sapiens
KANFDAQQFAGTWLLVAVGSACRF

SEQ ID NO: 501 - protein, 23 aa, Homo sapiens
RAEATTLHVAPQGTAMAVSTFRK

SEQ ID NO: 502 - protein, 15 aa, Homo sapiens
RDVVLTTTFVDDIKA

SEQ ID NO: 503 - protein, 15 aa, Homo sapiens
RRPWNVASLIYETKG

SEQ ID NO: 504 - protein, 10 aa, Homo sapiens
KISVIRPSKG

SEQ ID NO: 505 - protein, 11 aa, Homo sapiens
KVASYGVKPRY

SEQ ID NO: 506 - protein, 16 aa, Homo sapiens
RDFHINLFQVLPWLKE

SEQ ID NO: 507 - protein, 9 aa, Homo sapiens
RDLLYIGKD

SEQ ID NO: 508 - protein, 13 aa, Homo sapiens
RLEDSVTYHCSRG

SEQ ID NO: 509 - protein, 13 aa, Homo sapiens
RLPPTTTCQQQKE

SEQ ID NO: 510 - protein, 11 aa, Homo sapiens
KCLHPCVISRE

SEQ ID NO: 511 - protein, 11 aa, Homo sapiens
KIDVHLVPDRK

SEQ ID NO: 512 - protein, 16 aa, Homo sapiens
KSIDVACHPGYALPKA

SEQ ID NO: 513 - protein, 25 aa, Homo sapiens
KVSVLCQENYLIQEGEEITCKDGRW

SEQ ID NO: 514 - protein, 15 aa, Homo sapiens
KWSSPPQCEGLPCKS

SEQ ID NO: 515 - protein, 12 aa, Homo sapiens
RWQSIPLCVEKI

SEQ ID NO: 516 - protein, 19 aa, Homo sapiens
RYQIWTTVVDWIHPDLKRI

SEQ ID NO: 517 - protein, 32 aa, Homo sapiens
KAVLQLNEEGVDTAGSTGVTLNLTSKPIILRF

SEQ ID NO: 518 - protein, 17 aa, Homo sapiens
RGLASANVDFAFSLYKH

SEQ ID NO: 519 - protein, 22 aa, Homo sapiens
KTFPGFFSPMLGEFVSETESRG

SEQ ID NO: 520 - protein, 26 aa, Homo sapiens
KFDLVPVPTNLYGDFFTGDAYVILKT

SEQ ID NO: 521 - protein, 19 aa, Homo sapiens
KQTQVSVLPEGGETPLFKQ

SEQ ID NO: 522 - protein, 24 aa, Homo sapiens
RAQPVQVAEGSEPDGFWEALGGKA

SEQ ID NO: 523 - protein, 32 aa, Homo sapiens
RIEGSNKVPVDPATYGQFYGGDSYIILYNYRH

SEQ ID NO: 524 - protein, 14 aa, Homo sapiens
KFLVGPDGIPIMRW

SEQ ID NO: 525 - protein, 17 aa, Homo sapiens
KALPQPQNVTSLLGCTH

SEQ ID NO: 526 - protein, 32 aa, Homo sapiens
KSLGPNSCSANGPGLYLIHGPNLYCYSDVEKL

SEQ ID NO: 527 - protein, 30 aa, Homo sapiens
RDGWHSWPIAHQWPQGPSAVDAAFSWEEKL

SEQ ID NO: 528 - protein, 17 aa, Homo sapiens
RGECQAEGVLFFQGDRE

SEQ ID NO: 529 - protein, 29 aa, Homo sapiens
RGECQAEGVLFFQGDREWFWDLATGTMKE

SEQ ID NO: 530 - protein, 29 aa, Homo sapiens
RLEKEVGTPHGIILDSVDAAFICPGSSRL

SEQ ID NO: 531 - protein, 9 aa, Homo sapiens
RLWWLDLKS

SEQ ID NO: 532 - protein, 15 aa, Homo sapiens
RWKNFPSPVDAAFRQ

SEQ ID NO: 533 - protein, 30 aa, Homo sapiens
KDQVNTFDNIFIAPVGISTAMGMISLGLKG

SEQ ID NO: 534 - protein, 11 aa, Homo sapiens
KANVFVQLPRL

SEQ ID NO: 535 - protein, 16 aa, Homo sapiens
RLEALPNSLLAPLGRL

SEQ ID NO: 536 - protein, 9 aa, Homo sapiens
RLFQGLGKL

SEQ ID NO: 537 - protein, 17 aa, Homo sapiens
RNLIAAVAPGAFLGLKA

SEQ ID NO: 538 - protein, 13 aa, Homo sapiens
RTFTPQPPGLERL

SEQ ID NO: 539 - protein, 14 aa, Homo sapiens
KVTFQLTYEEVLKR

SEQ ID NO: 540 - protein, 15 aa, Homo sapiens
KVTFQLTYEEVLKRN

SEQ ID NO: 541 - protein, 39 aa, Homo sapiens
RGIEILNQVQESLPELSNHASILIMLTDGDPTEGVTDRS

SEQ ID NO: 542 - protein, 15 aa, Homo sapiens
RKAAISGENAGLVRA

SEQ ID NO: 543 - protein, 27 aa, Homo sapiens
KAGELEVFNGYFVHFFAPDNLDPIPKN

SEQ ID NO: 544 - protein, 13 aa, Homo sapiens
KFYNQVSTPLLRN

SEQ ID NO: 545 - protein, 13 aa, Homo sapiens
KVQFELHYQEVKW

SEQ ID NO: 546 - protein, 17 aa, Homo sapiens
RETAVDGELVVLYDVKR

SEQ ID NO: 547 - protein, 9 aa, Homo sapiens
RIYLQPGRL

SEQ ID NO: 548 - protein, 15 aa, Homo sapiens
RLWAYLTIEQLLEKR

SEQ ID NO: 549 - protein, 14 aa, Homo sapiens
KITFELVYEELLKR

SEQ ID NO: 550 - protein, 18 aa, Homo sapiens
KLQDRGPDVLTATVSGKL

SEQ ID NO: 551 - protein, 29 aa, Homo sapiens
KTGLLLLSDPDKVTIGLLFWDGRGEGLRL

SEQ ID NO: 552 - protein, 30 aa, Homo sapiens
RAISGGSIQIENGYFVHYFAPEGLTTMPKN

SEQ ID NO: 553 - protein, 17 aa, Homo sapiens
RANTVQEATFQMELPKK

SEQ ID NO: 554 - protein, 35 aa, Homo sapiens
RSFAAGIQALGGTNINDAMLMAVQLLDSSNQEERL

SEQ ID NO: 555 - protein, 12 aa, Homo sapiens
RVQGNDHSATRE

SEQ ID NO: 556 - protein, 15 aa, Homo sapiens
KITFELVYEELLKRR

SEQ ID NO: 557 - protein, 13 aa, Homo sapiens
KVTIGLLFWDGRG

SEQ ID NO: 558 - protein, 28 aa, Homo sapiens
RLWAYLTIQQLLEQTVSASDADQQALRN

SEQ ID NO: 559 - protein, 23 aa, Homo sapiens
KLFHTNFYDTVGTIQLINDHVKK

SEQ ID NO: 560 - protein, 13 aa, Homo sapiens
KENFLFLTPDCKS

SEQ ID NO: 561 - protein, 19 aa, Homo sapiens
KIYPTVNCQPLGMISLMKR

SEQ ID NO: 562 - protein, 20 aa, Homo sapiens
KKIYPTVNCQPLGMISLMKR

SEQ ID NO: 563 - protein, 23 aa, Homo sapiens
KSLWNGDTGECTDNAYIDIQLRI

SEQ ID NO: 564 - protein, 11 aa, Homo sapiens
KILGPLSYSKI

SEQ ID NO: 565 - protein, 31 aa, Homo sapiens
KEYGVVLAPDGSTVAVEPLLAGLEAGLQGRR

SEQ ID NO: 566 - protein, 34 aa, Homo sapiens
REGKEYGVVLAPDGSTVAVEPLLAGLEAGLQGRR

SEQ ID NO: 567 - protein, 27 aa, Homo sapiens
RQNGAALTSASILAQQVWGTLVLLQRL

SEQ ID NO: 568 - protein, 21 aa, Homo sapiens
KIAQLPLTGSMSIIFFLPLKV

SEQ ID NO: 569 - protein, 32 aa, Homo sapiens
RSSTSPTTNVLLSPLSVATALSALSLGAEQRT

SEQ ID NO: 570 - protein, 13 aa, Homo sapiens
KVAEYMDWILEKT

SEQ ID NO: 571 - protein, 15 aa, Homo sapiens
RCQFFSYATQTFHKA

SEQ ID NO: 572 - protein, 19 aa, Homo sapiens
RCLLFSFLPASSINDMEKR

SEQ ID NO: 573 - protein, 14 aa, Homo sapiens
RLVLLNAIYLSAKW

SEQ ID NO: 574 - protein, 16 aa, Homo sapiens
RNALFCLESAWNVAKE

SEQ ID NO: 575 - protein, 18 aa, Homo sapiens
RSNPVILNVLYGPDLPRI

SEQ ID NO: 576 - protein, 20 aa, Homo sapiens
KIAIIGAGIGGTSAAYYLRQ

SEQ ID NO: 577 - protein, 16 aa, Homo sapiens
KWYNLAIGSTCPWLKK

SEQ ID NO: 578 - protein, 13 aa, Homo sapiens
RTVAACNLPIVRG

SEQ ID NO: 579 - protein, 22 aa, Homo sapiens
RIVEGSDAEIGMSPWQVMLFRK

SEQ ID NO: 580 - protein, 23 aa, Homo sapiens
RRQECSIPVCGQDQVTVAMTPRS

SEQ ID NO: 581 - protein, 19 aa, Homo sapiens
RTFGSGEADCGLRPLFEKK

SEQ ID NO: 582 - protein, 25 aa, Homo sapiens
RLLNNWDVCADMVGTFTDTEDPAKF

SEQ ID NO: 583 - protein, 12 aa, Homo sapiens
RGYVIIKPLVWV

SEQ ID NO: 584 - protein, 26 aa, Homo sapiens
KVVLSSGSGPGLDLPLVLGLPLQLKL

SEQ ID NO: 585 - protein, 11 aa, Homo sapiens
KGFLLLASLRQ

SEQ ID NO: 586 - protein, 10 aa, Homo sapiens
KAVLHIGEKG

SEQ ID NO: 587 - protein, 17 aa, Homo sapiens
KFSISATYDLGATLLKM

SEQ ID NO: 588 - protein, 17 aa, Homo sapiens
KKELELQIGNALFIGKH

SEQ ID NO: 589 - protein, 16 aa, Homo sapiens
KMSSINADFAFNLYRR

SEQ ID NO: 590 - protein, 14 aa, Homo sapiens
RLTLLAPLNSVFKD

SEQ ID NO: 591 - protein, 15 aa, Homo sapiens
RGSPAINVAVHVFRK

SEQ ID NO: 592 - protein, 11 aa, Homo sapiens
KMPSHLMLARK

SEQ ID NO: 593 - protein, 10 aa, Homo sapiens
KELPEHTVKL

SEQ ID NO: 594 - protein, 29 aa, Homo sapiens
KEYANQFMWEYSTNYGQAPLSLLVSYTKS

SEQ ID NO: 595 - protein, 13 aa, Homo sapiens
KHLSLLTTLSNRV

SEQ ID NO: 596 - protein, 24 aa, Homo sapiens
KHQPQEFPTYVEPTNDEICEAFRK

SEQ ID NO: 597 - protein, 28 aa, Homo sapiens
KLAQKVPTADLEDVLPLAEDITNILSKC

SEQ ID NO: 598 - protein, 10 aa, Homo sapiens
KLCDNLSTKN

SEQ ID NO: 599 - protein, 9 aa, Homo sapiens
KLCMAALKH

SEQ ID NO: 600 - protein, 22 aa, Homo sapiens
KSCESNSPFPVHPGTAECCTKE

SEQ ID NO: 601 - protein, 23 aa, Homo sapiens
KSYLSMVGSCCTSASPTVCFLKE

SEQ ID NO: 602 - protein, 31 aa, Homo sapiens
KTAMDVFVCTYFMPAAQLPELPDVELPTNKD

SEQ ID NO: 603 - protein, 9 aa, Homo sapiens
KVLEPTLKS

SEQ ID NO: 604 - protein, 17 aa, Homo sapiens
RKFPSGTFEQVSQLVKE

SEQ ID NO: 605 - protein, 12 aa, Homo sapiens
RTHLPEVFLSKV

SEQ ID NO: 606 - protein, 9 aa, Homo sapiens
RTSALSAKS

SEQ ID NO: 607 - protein, 12 aa, Homo sapiens
RGQYCYELDEKA

SEQ ID NO: 608 - protein, 24 aa, Homo sapiens
RMDWLVPATCEPIQSVFFFSGDKY

SEQ ID NO: 609 - protein, 9 aa, Homo sapiens
RQPQFISRD

SEQ ID NO: 610 - protein, 9 aa, Homo sapiens
KHFQNLGKD

SEQ ID NO: 611 - protein, 14 aa, Homo sapiens
RRHPDLSIPELLRI

SEQ ID NO: 612 - protein, 13 aa, Homo sapiens
RTINPAVDHCCKT

SEQ ID NO: 613 - protein, 22 aa, Homo sapiens
RDYNLNDILLQLGIEEAFTSKA

SEQ ID NO: 614 - protein, 23 aa, Homo sapiens
RGTHVDLGLASANVDFAFSLYKQ

SEQ ID NO: 615 - protein, 28 aa, Homo sapiens
KGFPIKEDFLEQSEQLFGAKPVSLTGKQ

SEQ ID NO: 616 - protein, 20 aa, Homo sapiens
RQLTSGPNQEQVSPLTLLKL

SEQ ID NO: 617 - protein, 26 aa, Homo sapiens
RAQLVPLPPSTYVEFTVSGTDCVAKE

SEQ ID NO: 618 - protein, 14 aa, Homo sapiens
KDPTFIPAPIQAKT

SEQ ID NO: 619 - protein, 11 aa, Homo sapiens
RFMQAVTGWKT

SEQ ID NO: 620 - protein, 12 aa, Homo sapiens
KANRPFLVFIRE

SEQ ID NO: 621 - protein, 17 aa, Homo sapiens
KGDDITMVLILPKPEKS

SEQ ID NO: 622 - protein, 13 aa, Homo sapiens
RDIPMNPMCIYRS

SEQ ID NO: 623 - protein, 14 aa, Homo sapiens
KKLVPFATELHERL

SEQ ID NO: 624 - protein, 19 aa, Homo sapiens
KSLAELGGHLDQQVEEFRR

SEQ ID NO: 625 - protein, 17 aa, Homo sapiens
KALYWVNGQVPDGVSKV

SEQ ID NO: 626 - protein, 9 aa, Homo sapiens
KFIIPGLKL

SEQ ID NO: 627 - protein, 20 aa, Homo sapiens
KFSVPAGIVIPSFQALTARF

SEQ ID NO: 628 - protein, 17 aa, Homo sapiens
KIEGNLIFDPNNYLPKE

SEQ ID NO: 629 - protein, 28 aa, Homo sapiens
KLNDLNSVLVMPTFHVPFTDLQVPSCKL

SEQ ID NO: 630 - protein, 16 aa, Homo sapiens
KVELEVPQLCSFILKT

SEQ ID NO: 631 - protein, 18 aa, Homo sapiens
KVNWEEEAASGLLTSLKD

SEQ ID NO: 632 - protein, 17 aa, Homo sapiens
RATLYALSHAVNNYHKT

SEQ ID NO: 633 - protein, 12 aa, Homo sapiens
RTGISPLALIKG

SEQ ID NO: 634 - protein, 16 aa, Homo sapiens
RTLQGIPQMIGEVIRK

SEQ ID NO: 635 - protein, 18 aa, Homo sapiens
KDALSSVQESQVAQQARG

SEQ ID NO: 636 - protein, 15 aa, Homo sapiens
RDGWQWFWSPSTFRG

SEQ ID NO: 637 - protein, 18 aa, Homo sapiens
KVQAAVGTSAAPVPSDNH

SEQ ID NO: 638 - protein, 9 aa, Homo sapiens
RWELALGRF

SEQ ID NO: 639 - protein, 24 aa, Homo sapiens
KSNFLNCYVSGFHPSDIEVDLLKN

SEQ ID NO: 640 - protein, 12 aa, Homo sapiens
RGGHCVALCTRG

SEQ ID NO: 641 - protein, 22 aa, Homo sapiens
RLVDFYVMPVVNVDGYDYSWKK

SEQ ID NO: 642 - protein, 29 aa, Homo sapiens
RYTHGHGSETLYLAPGGGDDWIYDLGIKY

SEQ ID NO: 643 - protein, 18 aa, Homo sapiens
KLSNNALSGLPQGVFGKL

SEQ ID NO: 644 - protein, 29 aa, Homo sapiens
KTLNLAQNLLAQLPEELFHPLTSLQTLKL

SEQ ID NO: 645 - protein, 11 aa, Homo sapiens
RWLNVQLSPRQ

SEQ ID NO: 646 - protein, 32 aa, Homo sapiens
KGDSVVWYLFSAGNEADVHGIYFSGNTYLWRG

SEQ ID NO: 647 - protein, 12 aa, Homo sapiens
KMYYSAVDPTKD

SEQ ID NO: 648 - protein, 25 aa, Homo sapiens
RGPEEEHLGILGPVIWAEVGDTIRV

SEQ ID NO: 649 - protein, 39 aa, Homo sapiens
RSGAGTEDSACIPWAYYSTVDQVKDLYSGLIGPLIVCRR

SEQ ID NO: 650 - protein, 13 aa, Homo sapiens
KIFFPGVSEFGKE

SEQ ID NO: 651 - protein, 23 aa, Homo sapiens
RAILQSGSFNAPWAVTSLYEARN

SEQ ID NO: 652 - protein, 19 aa, Homo sapiens
RVLQGVLPALPQVVCNYRD

SEQ ID NO: 653 - protein, 16 aa, Homo sapiens
RISLLLIESWLEPVRF

SEQ ID NO: 654 - protein, 20 aa, Homo sapiens
RLHEAFSPVSYQHDLALLRL

SEQ ID NO: 655 - protein, 20 aa, Homo sapiens
RTTLSGAPCQPWASEATYRN

SEQ ID NO: 656 - protein, 29 aa, Homo sapiens
KGLFQVVSGGMVLQLQQGDQVWVEKDPKK

SEQ ID NO: 657 - protein, 12 aa, Homo sapiens
KVLNYVDWIKKE

SEQ ID NO: 658 - protein, 18 aa, Homo sapiens
KSNALDIIFQTDLTGQKK

SEQ ID NO: 659 - protein, 21 aa, Homo sapiens
KEGAIHREELVYELNPLDHRG

SEQ ID NO: 660 - protein, 11 aa, Homo sapiens
KITQVLHFTKD

SEQ ID NO: 661 - protein, 11 aa, Homo sapiens
KSHALQLNNRQ

SEQ ID NO: 662 - protein, 20 aa, Homo sapiens
RAVGSGATFSHYYYMILSRG

SEQ ID NO: 663 - protein, 16 aa, Homo sapiens
REPFLSCCQFAESLRK

SEQ ID NO: 664 - protein, 19 aa, Homo sapiens
RGHLFLQTDQPIYNPGQRV

SEQ ID NO: 665 - protein, 15 aa, Homo sapiens
RGLEEELQFSLGSKI

SEQ ID NO: 666 - protein, 15 aa, Homo sapiens
RGSFEFPVGDAVSKV

SEQ ID NO: 667 - protein, 19 aa, Homo sapiens
RLLATLCSAEVCQCAEGKC

SEQ ID NO: 668 - protein, 24 aa, Homo sapiens
RVQQPDCREPFLSCCQFAESLRKK

SEQ ID NO: 669 - protein, 16 aa, Homo sapiens
RYIYGKPVQGVAYVRF

SEQ ID NO: 670 - protein, 13 aa, Homo sapiens
KITHYNYLILSKG

SEQ ID NO: 671 - protein, 17 aa, Homo sapiens
RENSLYLTAFTVIGIRK

SEQ ID NO: 672 - protein, 12 aa, Homo sapiens
RKAFDICPLVKI

SEQ ID NO: 673 - protein, 26 aa, Homo sapiens
RVDDGVASFVLNLPSGVTVLEFNVKT

SEQ ID NO: 674 - protein, 30 aa, Homo sapiens
KTFSEWLESVKENPAVIDFELAPIVDLVRN

SEQ ID NO: 675 - protein, 33 aa, Homo sapiens
RIFDDFGTHYFTSGSLGGVYDLLYQFSSEELKN

SEQ ID NO: 676 - protein, 17 aa, Homo sapiens
KELSHLPSLYDYSAYRR

SEQ ID NO: 677 - protein, 19 aa, Homo sapiens
RRYSAWAESVTNLPQVIKQ

SEQ ID NO: 678 - protein, 22 aa, Homo sapiens
KVEPLYELVTATDFAYSSTVRQ

SEQ ID NO: 679 - protein, 13 aa, Homo sapiens
RSLMLHYEFLQRV

SEQ ID NO: 680 - protein, 19 aa, Homo sapiens
KYGFCEAADQFHVLDEVRR

SEQ ID NO: 681 - protein, 10 aa, Homo sapiens
RFLQEQGHRA

SEQ ID NO: 682 - protein, 12 aa, Homo sapiens
RKLDGICWQVRQ

SEQ ID NO: 683 - protein, 17 aa, Homo sapiens
RSLPVSDSVLSGFEQRV

SEQ ID NO: 684 - protein, 28 aa, Homo sapiens
RGTVIDVTDFVNWASSINDAPVLISQKL

SEQ ID NO: 685 - protein, 31 aa, Homo sapiens
KNPREDYLDVYVFGVGPLVNQVNINALASKK

SEQ ID NO: 686 - protein, 14 aa, Homo sapiens
RGDSGGPLIVHKRS

SEQ ID NO: 687 - protein, 27 aa, Homo sapiens
RHVIILMTDGLHNMGGDPITVIDEIRD

SEQ ID NO: 688 - protein, 32 aa, Homo sapiens
RKNPREDYLDVYVFGVGPLVNQVNINALASKK

SEQ ID NO: 689 - protein, 13 aa, Homo sapiens
KSCDIPVFMNART

SEQ ID NO: 690 - protein, 28 aa, Homo sapiens
KSPPEISHGVVAHMSDSYQYGEEVTYKC

SEQ ID NO: 691 - protein, 21 aa, Homo sapiens
KTDCLSLPSFENAIPMGEKKD

SEQ ID NO: 692 - protein, 16 aa, Homo sapiens
KRAQLGDLPWQVAIKD

SEQ ID NO: 693 - protein, 12 aa, Homo sapiens
KSLECLHPGTKF

SEQ ID NO: 694 - protein, 18 aa, Homo sapiens
RTMGYQDFADVVCYTQKA

SEQ ID NO: 695 - protein, 12 aa, Homo sapiens
RELLALIQLERE

SEQ ID NO: 696 - protein, 20 aa, Homo sapiens
RVPEARPNSMVVEHPEFLKA

SEQ ID NO: 697 - protein, 9 aa, Homo sapiens
RLFWEPMKV

SEQ ID NO: 698 - protein, 14 aa, Homo sapiens
RDVRDYFMPCPGRG

SEQ ID NO: 699 - protein, 23 aa, Homo sapiens
KDALENIDPATQMMILNCIYFKG

SEQ ID NO: 700 - protein, 27 aa, Homo sapiens
KGLIKDALENIDPATQMMILNCIYFKG

SEQ ID NO: 701 - protein, 11 aa, Homo sapiens
KQFPILLDFKT

SEQ ID NO: 702 - protein, 12 aa, Homo sapiens
RAFWLDVSHNRL

SEQ ID NO: 703 - protein, 27 aa, Homo sapiens
KADVQAHGEGQEFSITCLVDEEEMKKL

SEQ ID NO: 704 - protein, 21 aa, Homo sapiens
KILGDMQPGDYFDLVLFGTRV

SEQ ID NO: 705 - protein, 15 aa, Homo sapiens
KNVVFVIDISGSMRG

SEQ ID NO: 706 - protein, 25 aa, Homo sapiens
KTAFISDFAVTADGNAFIGDIKDKV

SEQ ID NO: 707 - protein, 12 aa, Homo sapiens
RGHMLENHVERL

SEQ ID NO: 708 - protein, 15 aa, Homo sapiens
RLWAYLTIQELLAKR

SEQ ID NO: 709 - protein, 12 aa, Homo sapiens
RNHMQYEIVIKV

SEQ ID NO: 710 - protein, 15 aa, Homo sapiens
KAHVSFKPTVAQQRI

SEQ ID NO: 711 - protein, 27 aa, Homo sapiens
KENIQDNISLFSLGMGFDVDYDFLKRL

SEQ ID NO: 712 - protein, 17 aa, Homo sapiens
KHLEVDVWVIEPQGLRF

SEQ ID NO: 713 - protein, 16 aa, Homo sapiens
KLWAYLTINQLLAERS

SEQ ID NO: 714 - protein, 17 aa, Homo sapiens
RAEDHFSVIDFNQNIRT

SEQ ID NO: 715 - protein, 22 aa, Homo sapiens
RFLHVPDTFEGHFDGVPVISKG

SEQ ID NO: 716 - protein, 10 aa, Homo sapiens
KILDDLSPRD

SEQ ID NO: 717 - protein, 13 aa, Homo sapiens
KIPKPEASFSPRR

SEQ ID NO: 718 - protein, 18 aa, Homo sapiens
KSPEQQETVLDGNLIIRY

SEQ ID NO: 719 - protein, 31 aa, Homo sapiens
RFSSHVGGTLGQFYQEVLWGSPAASDDGRRT

SEQ ID NO: 720 - protein, 14 aa, Homo sapiens
RGPDVLTATVSGKL

SEQ ID NO: 721 - protein, 18 aa, Homo sapiens
RNMEQFQVSVSVAPNAKI

SEQ ID NO: 722 - protein, 21 aa, Homo sapiens
RRLDYQEGPPGVEISCWSVEL

SEQ ID NO: 723 - protein, 12 aa, Homo sapiens
KIVDLVSELKKD

SEQ ID NO: 724 - protein, 14 aa, Homo sapiens
RVGSALFLSHNLKF

SEQ ID NO: 725 - protein, 13 aa, Homo sapiens
KTVGSDTFYSFKY

SEQ ID NO: 726 - protein, 21 aa, Homo sapiens
RDIPTNSPELEETLTHTITKL

SEQ ID NO: 727 - protein, 9 aa, Homo sapiens
RVQVVAGKK

SEQ ID NO: 728 - protein, 10 aa, Homo sapiens
RFNALQYLRL

SEQ ID NO: 729 - protein, 19 aa, Homo sapiens
KVIPGPPALTLVPAELVRI

SEQ ID NO: 730 - protein, 23 aa, Homo sapiens
KITGTMPPLPLEATGLALSSLRL

SEQ ID NO: 731 - protein, 17 aa, Homo sapiens
KEFTEAFLGCPAIHPRC

SEQ ID NO: 732 - protein, 33 aa, Homo sapiens
RRVINLPLDSMAAPWETGDTFPDVVAIAPDVRA

SEQ ID NO: 733 - protein, 21 aa, Homo sapiens
RGVFFSVNSWTPDSMSFIYKA

SEQ ID NO: 734 - protein, 19 aa, Homo sapiens
KEIPDEISILLLGVAHFKG

SEQ ID NO: 735 - protein, 12 aa, Homo sapiens
KTVQAVLTVPKL

SEQ ID NO: 736 - protein, 30 aa, Homo sapiens
RALYYDLISSPDIHGTYKELLDTVTAPQKN

SEQ ID NO: 737 - protein, 14 aa, Homo sapiens
RDTDTGALLFIGKI

SEQ ID NO: 738 - protein, 16 aa, Homo sapiens
RELRPWCFTTDPNKRW

SEQ ID NO: 739 - protein, 23 aa, Homo sapiens
RTECFITGWGETQGTFGAGLLKE

SEQ ID NO: 740 - protein, 16 aa, Homo sapiens
KGTHCNQVEVIATLKD

SEQ ID NO: 741 - protein, 13 aa, Homo sapiens
KAVGYLITGYQRQ

SEQ ID NO: 742 - protein, 29 aa, Homo sapiens
RAVDQSVLLMKPEAELSVSSVYNLLTVKD

SEQ ID NO: 743 - protein, 16 aa, Homo sapiens
RIQHPFTVEEFVLPKF

SEQ ID NO: 744 - protein, 15 aa, Homo sapiens
RNELIPLIYLENPRR

SEQ ID NO: 745 - protein, 14 aa, Homo sapiens
RAFIQLWAFDAVKG

SEQ ID NO: 746 - protein, 19 aa, Homo sapiens
KGFGGLTGQIVAALSTAKY

SEQ ID NO: 747 - protein, 11 aa, Homo sapiens
KYGFYTHVFRL

SEQ ID NO: 748 - protein, 31 aa, Homo sapiens
KKDPEGLFLQDNIVAEFSVDETGQMSATAKG

SEQ ID NO: 749 - protein, 24 aa, Homo sapiens
KAQWANPFDPSKTEDSSSFLIDKT

SEQ ID NO: 750 - protein, 11 aa, Homo sapiens
KGWVDLFVPKF

SEQ ID NO: 751 - protein, 11 aa, Homo sapiens
RSFMLLILERS

SEQ ID NO: 752 - protein, 22 aa, Homo sapiens
KEFSHLGKEDFTSLSLVLYSRK

SEQ ID NO: 753 - protein, 25 aa, Homo sapiens
KHQPQEFPTYVEPTNDEICEAFRKD

SEQ ID NO: 754 - protein, 24 aa, Homo sapiens
KVPTADLEDVLPLAEDITNILSKC

SEQ ID NO: 755 - protein, 10 aa, Homo sapiens
KAVRPGYPKL

SEQ ID NO: 756 - protein, 18 aa, Homo sapiens
KEIPAWVPFDPAAQITKQ

SEQ ID NO: 757 - protein, 12 aa, Homo sapiens
RNLAVSQVVHKA

SEQ ID NO: 758 - protein, 14 aa, Homo sapiens
KAAISGENAGLVRA

SEQ ID NO: 759 - protein, 23 aa, Homo sapiens
KTAFISDFAVTADGNAFIGDIKD

SEQ ID NO: 760 - protein, 9 aa, Homo sapiens
KVTYDVSRD

SEQ ID NO: 761 - protein, 12 aa, Homo sapiens
REVAFDLEIPKT

SEQ ID NO: 762 - protein, 8 aa, Homo sapiens
KTAGLVRS

SEQ ID NO: 763 - protein, 12 aa, Homo sapiens
RSLAPTAAAKRR

SEQ ID NO: 764 - protein, 12 aa, Homo sapiens
KEVSFDVELPKT

SEQ ID NO: 765 - protein, 8 aa, Homo sapiens
KIQENVRN

SEQ ID NO: 766 - protein, 9 aa, Homo sapiens
RALDLSLKY

SEQ ID NO: 767 - protein, 21 aa, Homo sapiens
RLIQDAVTGLTVNGQITGDKR

SEQ ID NO: 768 - protein, 11 aa, Homo sapiens
KSSFVAPLEKS

SEQ ID NO: 769 - protein, 13 aa, Homo sapiens
KELLDTVTAPQKN

SEQ ID NO: 770 - protein, 9 aa, Homo sapiens
KFQLPGQKL

SEQ ID NO: 771 - protein, 27 aa, Homo sapiens
RDLYHYITSYVVDGEIIIYGPAYSGRE

SEQ ID NO: 772 - protein, 11 aa, Homo sapiens
KLFIPQITPKH

SEQ ID NO: 773 - protein, 15 aa, Homo sapiens
NSATGEESSTSLTIR

SEQ ID NO: 774 - protein, 18 aa, Homo sapiens
KFQQSGQNLFIPQITTKH

SEQ ID NO: 775 - protein, 9 aa, Homo sapiens
IHPSYTNYR

SEQ ID NO: 776 - protein, 8 aa, Homo sapiens
FQLSETNR

SEQ ID NO: 777 - protein, 16 aa, Homo sapiens
VSAPSGTGHLPGLNPL

SEQ ID NO: 778 - protein, 12 aa, Homo sapiens
EDAGSYTLHIVK

SEQ ID NO: 779 - protein, 11 aa, Homo sapiens
RTLFIFGVTKY

SEQ ID NO: 780 - protein, 18 aa, Homo sapiens
NYTYIWWLNGQSLPVSPR

SEQ ID NO: 781 - protein, 13 aa, Homo sapiens
GVTGYFTFNLYLK

SEQ ID NO: 782 - protein, 16 aa, Homo sapiens
SNPVTLNVLYGPDLPR

SEQ ID NO: 783 - protein, 20 aa, Homo sapiens
DVLLLVHNLPQNLTGHIWYK

SEQ ID NO: 784 - protein, 8 aa, Homo sapiens
YGPAYSGR

SEQ ID NO: 785 - protein, 8 aa, Homo sapiens
LQLSETNR

SEQ ID NO: 786 - protein, 10 aa, Homo sapiens
KLFIPQITRN

SEQ ID NO: 787 - protein, 16 aa, Homo sapiens
KLPIPYITINNLNPRE

SEQ ID NO: 788 - protein, 22 aa, Homo sapiens
SENYTYIWWLNGQSLPVSPGVK

SEQ ID NO: 789 - protein, 9 aa, Homo sapiens
ILILPSVTR

SEQ ID NO: 790 - protein, 13 aa, Homo sapiens
KAQWANPFDPSKT

SEQ ID NO: 791 - protein, 8 aa, Homo sapiens
KFLNDVKT

SEQ ID NO: 792 - protein, 12 aa, Homo sapiens
KNALALFVLPKE

SEQ ID NO: 793 - protein, 12 aa, Homo sapiens
RDFNQFSSGEKN

SEQ ID NO: 794 - protein, 10 aa, Homo sapiens
KGYQELLEKC

SEQ ID NO: 795 - protein, 9 aa, Homo sapiens
KGEEELQKY

SEQ ID NO: 796 - protein, 9 aa, Homo sapiens
KFIYEIARR

SEQ ID NO: 797 - protein, 17 aa, Homo sapiens
RHPFLYAPTILLWAARY

SEQ ID NO: 798 - protein, 11 aa, Homo sapiens
RTFQAITVTKL

SEQ ID NO: 799 - protein, 8 aa, Homo sapiens
KLTTLERG

SEQ ID NO: 800 - protein, 13 aa, Homo sapiens
RHPQLAVSVILRV

SEQ ID NO: 801 - protein, 18 aa, Homo sapiens
KLGEYYLQNAFLVAYTKK

SEQ ID NO: 802 - protein, 9 aa, Homo sapiens
RILPSVPKD

SEQ ID NO: 803 - protein, 18 aa, Homo sapiens
KAEHPTWGDEQLFQTTRL

SEQ ID NO: 804 - protein, 11 aa, Homo sapiens
RLILIGETIKI

SEQ ID NO: 805 - protein, 10 aa, Homo sapiens
RLQPFNEYRK

SEQ ID NO: 806 - protein, 14 aa, Homo sapiens
ELIEELVNITQNQK

SEQ ID NO: 807 - protein, 19 aa, Homo sapiens
LIQDAVTGLTVNGQITGDK

SEQ ID NO: 808 - protein, 8 aa, Homo sapiens
QALEEFQK

SEQ ID NO: 809 - protein, 10 aa, Homo sapiens
DAGLSWGSAR

SEQ ID NO: 810 - protein, 7 aa, Homo sapiens
VFQFLEK

SEQ ID NO: 811 - protein, 7 aa, Homo sapiens
VQTAHFK

SEQ ID NO: 812 - protein, 9 aa, Homo sapiens
SDLEVAHYK

SEQ ID NO: 813 - protein, 14 aa, Homo sapiens
VSEADSSNADWVTK

SEQ ID NO: 814 - protein, 9 aa, Homo sapiens
LPNNVLQEK

SEQ ID NO: 815 - protein, 10 aa, Homo sapiens
TTSDGGYSFK

SEQ ID NO: 816 - protein, 11 aa, Homo sapiens
YENYTSSFFIR

SEQ ID NO: 817 - protein, 8 aa, Homo sapiens
AVLHIGEK

SEQ ID NO: 818 - protein, 19 aa, Homo sapiens
GLQYAAQEGLLALQSELLR

SEQ ID NO: 819 - protein, 11 aa, Homo sapiens
QLYGDTGVLGR

SEQ ID NO: 820 - protein, 9 aa, Homo sapiens
ELPQSIVYK

SEQ ID NO: 821 - protein, 8 aa, Homo sapiens
NIQSVNVK

SEQ ID NO: 822 - protein, 16 aa, Homo sapiens
TGVAVNKPAEFTVDAK

SEQ ID NO: 823 - protein, 21 aa, Homo sapiens
HELTDEELQSLFTNFANVVDK

SEQ ID NO: 824 - protein, 23 aa, Homo sapiens
TEFLSNYLTNVDDITLVPGTLGR

SEQ ID NO: 825 - protein, 7 aa, Homo sapiens
IAIDLFK

SEQ ID NO: 826 - protein, 10 aa, Homo sapiens
TVQAVLTVPK

SEQ ID NO: 827 - protein, 11 aa, Homo sapiens
LIENGYFHPVK

SEQ ID NO: 828 - protein, 7 aa, Homo sapiens
FLPCENK

SEQ ID NO: 829 - protein, 17 aa, Homo sapiens
HPWIVHWDQLPQYQLNR

SEQ ID NO: 830 - protein, 10 aa, Homo sapiens
QGHNSVFLIK

SEQ ID NO: 831 - protein, 7 aa, Homo sapiens
HFQNLGK

SEQ ID NO: 832 - protein, 16 aa, Homo sapiens
IAPQLSTEELVSLGEK

SEQ ID NO: 833 - protein, 10 aa, Homo sapiens
DADPDTFFAK

SEQ ID NO: 834 - protein, 10 aa, Homo sapiens
VNHVTLSQPK

SEQ ID NO: 835 - protein, 10 aa, Homo sapiens
HYGGLTGLNK

SEQ ID NO: 836 - protein, 13 aa, Homo sapiens
NCSFSIIYPVVIK

SEQ ID NO: 837 - protein, 22 aa, Homo sapiens
AQPVQVAEGSEPDGFWEALGGK

SEQ ID NO: 838 - protein, 9 aa, Homo sapiens
LDFHFSSDR

SEQ ID NO: 839 - protein, 8 aa, Homo sapiens
TLNAYDHR

SEQ ID NO: 840 - protein, 14 aa, Homo sapiens
EVFSKPISWEELLQ

SEQ ID NO: 841 - protein, 11 aa, Homo sapiens
NFPSPVDAAFR

SEQ ID NO: 842 - protein, 9 aa, Homo sapiens
TLFIFGVTK

SEQ ID NO: 843 - protein, 9 aa, Homo sapiens
YYGYTGAFR

SEQ ID NO: 844 - protein, 7 aa, Homo sapiens
QVFAVQR

SEQ ID NO: 845 - protein, 10 aa, Homo sapiens
DFNQFSSGEK

SEQ ID NO: 846 - protein, 13 aa, Homo sapiens
SVSLPSLDPASAK

SEQ ID NO: 847 - protein, 9 aa, Homo sapiens
GNGLTWAEK

SEQ ID NO: 848 - protein, 22 aa, Homo sapiens
GAVHVVVAETDYQSFAVLYLER

SEQ ID NO: 849 - protein, 14 aa, Homo sapiens
TSESTGSLPSPFLR

SEQ ID NO: 850 - protein, 12 aa, Homo sapiens
YISPDQLADLYK

SEQ ID NO: 851 - protein, 10 aa, Homo sapiens
ESDTSYVSLK

SEQ ID NO: 852 - protein, 8 aa, Homo sapiens
ILDDLSPR

SEQ ID NO: 853 - protein, 11 aa, Homo sapiens
SGVDLADSNQK

SEQ ID NO: 854 - protein, 12 aa, Homo sapiens
DTDTGALLFIGK

SEQ ID NO: 855 - protein, 9 aa, Homo sapiens
HYFIAAVER

SEQ ID NO: 856 - protein, 10 aa, Homo sapiens
DLHLSDVFLK

SEQ ID NO: 857 - protein, 12 aa, Homo sapiens
DPTFIPAPIQAK

SEQ ID NO: 858 - protein, 7 aa, Homo sapiens
AGITIPR

SEQ ID NO: 859 - protein, 9 aa, Homo sapiens
IAQYYYTFK

SEQ ID NO: 860 - protein, 10 aa, Homo sapiens
YNSQLLSFVR

SEQ ID NO: 861 - protein, 19 aa, Homo sapiens
ANDQYLTAAALHNLDEAVK

SEQ ID NO: 862 - protein, 9 aa, Homo sapiens
FQSVFTVTR

SEQ ID NO: 863 - protein, 14 aa, Homo sapiens
LQVNTPLVGASLLR

SEQ ID NO: 864 - protein, 12 aa, Homo sapiens
DEIPHNDIALLK

SEQ ID NO: 865 - protein, 10 aa, Homo sapiens
HATLSLSIPR

SEQ ID NO: 866 - protein, 10 aa, Homo sapiens
TGISPLALIK

SEQ ID NO: 867 - protein, 7 aa, Homo sapiens
ILPSVPK

SEQ ID NO: 868 - protein, 12 aa, Homo sapiens
LPATEKPVLLSK

SEQ ID NO: 869 - protein, 11 aa, Homo sapiens
TFLTVYWTPER

SEQ ID NO: 870 - protein, 16 aa, Homo sapiens
GDTYPAELYITGSILR

SEQ ID NO: 871 - protein, 13 aa, Homo sapiens
SLDFTELDVAAEK

SEQ ID NO: 872 - protein, 14 aa, Homo sapiens
VELAPLPSWQPVGK

SEQ ID NO: 873 - protein, 7 aa, Homo sapiens
GPGEDFR

SEQ ID NO: 874 - protein, 9 aa, Homo sapiens
ILNIFGVIK

SEQ ID NO: 875 - protein, 15 aa, Homo sapiens
ISQGEADINIAFYQR

SEQ ID NO: 876 - protein, 8 aa, Homo sapiens
FTITAGSK

SEQ ID NO: 877 - protein, 7 aa, Homo sapiens
ILDGGNK

SEQ ID NO: 878 - protein, 13 aa, Homo sapiens
FSLVSGWGQLLDR

SEQ ID NO: 879 - protein, 9 aa, Homo sapiens
SDGAKPGPR

SEQ ID NO: 880 - protein, 6 aa, Homo sapiens
QDLGWK

SEQ ID NO: 881 - protein, 7 aa, Homo sapiens
SILFLGK

SEQ ID NO: 882 - protein, 21 aa, Homo sapiens
IEVNESGTVASSSTAVIVSAR

SEQ ID NO: 883 - protein, 20 aa, Homo sapiens
LLAPSDSPEWLSFDVTGVVR

SEQ ID NO: 884 - protein, 8 aa, Homo sapiens
IEVIITLK

SEQ ID NO: 885 - protein, 7 aa, Homo sapiens
DYWSTVK

SEQ ID NO: 886 - protein, 12 aa, Homo sapiens
WILTAAHTLYPK

SEQ ID NO: 887 - protein, 12 aa, Homo sapiens
SPEAEDPLGVER

SEQ ID NO: 888 - protein, 16 aa, Homo sapiens
SGAQATWTELPWPHEK

SEQ ID NO: 889 - protein, 7 aa, Homo sapiens
YSHYNER

SEQ ID NO: 890 - protein, 20 aa, Homo sapiens
EVPLSALTNILSAQLISHWK

SEQ ID NO: 891 - protein, 22 aa, Homo sapiens
AALAAFNAQNNGSNFQLEEISR

SEQ ID NO: 892 - protein, 20 aa, Homo sapiens
IVLSLDVPIGLLQILLEQAR

SEQ ID NO: 893 - protein, 18 aa, Homo sapiens
ENPAVIDFELAPIVDLVR

SEQ ID NO: 894 - protein, 11 aa, Homo sapiens
NVNQSLLELHK

SEQ ID NO: 895 - protein, 9 aa, Homo sapiens
EIGELYLPK

SEQ ID NO: 896 - protein, 17 aa, Homo sapiens
NKPGVYTDVAYYLAWIR

SEQ ID NO: 897 - protein, 13 aa, Homo sapiens
QNYHQDSEAAINR

SEQ ID NO: 898 - protein, 6 aa, Homo sapiens
VTFEYR

SEQ ID NO: 899 - protein, 9 aa, Homo sapiens
DLPHITVDR

SEQ ID NO: 900 - protein, 19 aa, Homo sapiens
GSLVQASEANLQAAQDFVR

SEQ ID NO: 901 - protein, 5 aa, Homo sapiens
FLYHK

SEQ ID NO: 902 - protein, 8 aa, Homo sapiens
LQDAGVYR

SEQ ID NO: 903 - protein, 8 aa, Homo sapiens
INPASLDK

SEQ ID NO: 904 - protein, 8 aa, Homo sapiens
LEEHYELR

SEQ ID NO: 905 - protein, 11 aa, Homo sapiens
TSDQIHFFFAK

SEQ ID NO: 906 - protein, 11 aa, Homo sapiens
ATLSAAPSNPR

SEQ ID NO: 907 - protein, 13 aa, Homo sapiens
EANQSTLENFLER

SEQ ID NO: 908 - protein, 14 aa, Homo sapiens
GQQPADVTGTALPR

SEQ ID NO: 909 - protein, 12 aa, Homo sapiens
GEVTYTTSQVSK

SEQ ID NO: 910 - protein, 11 aa, Homo sapiens
SLQAFVAVAAR

SEQ ID NO: 911 - protein, 15 aa, Homo sapiens
GPEDQDISISFAWDK

SEQ ID NO: 912 - protein, 12 aa, Homo sapiens
YVVISQGLDKPR

SEQ ID NO: 913 - protein, 15 aa, Homo sapiens
GTAEWLSFDVTDTVR

SEQ ID NO: 914 - protein, 19 aa, Homo sapiens
AHQLAIDTYQEFEETYIPK

SEQ ID NO: 915 - protein, 10 aa, Homo sapiens
TAVTANLDIR

SEQ ID NO: 916 - protein, 16 aa, Homo sapiens
WSAGLTSSQVDLYIPK

SEQ ID NO: 917 - protein, 7 aa, Homo sapiens
QINSYVK

SEQ ID NO: 918 - protein, 12 aa, Homo sapiens
GFQALGDAADIR

SEQ ID NO: 919 - protein, 6 aa, Homo sapiens
NEIWYR

SEQ ID NO: 920 - protein, 7 aa, Homo sapiens
VLEPTLK

SEQ ID NO: 921 - protein, 11 aa, Homo sapiens
ALNSIIDVYHK

SEQ ID NO: 922 - protein, 25 aa, Homo sapiens
ETPEGAEAKPWYEPIYLGGVFQLEK

SEQ ID NO: 923 - protein, 10 aa, Homo sapiens
LNIGYIEDLK

SEQ ID NO: 924 - protein, 10 aa, Homo sapiens
DIPHWLNPTR

SEQ ID NO: 925 - protein, 17 aa, Homo sapiens
NEIVFPAGILQAPFYTR

SEQ ID NO: 926 - protein, 16 aa, Homo sapiens
AEHPTWGDEQLFQTTR

SEQ ID NO: 927 - protein, 14 aa, Homo sapiens
SWNEPLYHLVTEVR

SEQ ID NO: 928 - protein, 11 aa, Homo sapiens
IPKPEASFSPR

SEQ ID NO: 929 - protein, 11 aa, Homo sapiens
DDLYVSDAFHK

SEQ ID NO: 930 - protein, 26 aa, Homo sapiens
QRPPDLDTSSNAVDLLFFTDESGDSR

SEQ ID NO: 931 - protein, 16 aa, Homo sapiens
GQVPENEANVVITTLK

SEQ ID NO: 932 - protein, 18 aa, Homo sapiens
FTGSQPFGQGVEHATANK

SEQ ID NO: 933 - protein, 18 aa, Homo sapiens
LEPLYSASGPGLRPLVIK

SEQ ID NO: 934 - protein, 14 aa, Homo sapiens
IQHPFTVEEFVLPK

SEQ ID NO: 935 - protein, 8 aa, Homo sapiens
TEQAAVAR

SEQ ID NO: 936 - protein, 13 aa, Homo sapiens
LFYADHPFIFLVR

SEQ ID NO: 937 - protein, 8 aa, Homo sapiens
TSYQVYSK

SEQ ID NO: 938 - protein, 13 aa, Homo sapiens
NVIQISNDLENLR

SEQ ID NO: 939 - protein, 23 aa, Homo sapiens
AFLEVNEEGSEAAASTAVVIAGR

SEQ ID NO: 940 - protein, 18 aa, Homo sapiens
LHEAFSPVSYQHDLALLR

SEQ ID NO: 941 - protein, 18 aa, Homo sapiens
GPITSAAELNDPQSILLR

SEQ ID NO: 942 - protein, 14 aa, Homo sapiens
AVDIPGLEAATPYR

SEQ ID NO: 943 - protein, 10 aa, Homo sapiens
VPLALFALNR

SEQ ID NO: 944 - protein, 9 aa, Homo sapiens
VVGGLVALR

SEQ ID NO: 945 - protein, 11 aa, Homo sapiens
NHYTESISVAK

SEQ ID NO: 946 - protein, 24 aa, Homo sapiens
VVLSSGSGPGLDLPLVLGLPLQLK

SEQ ID NO: 947 - protein, 22 aa, Homo sapiens
ALALPPLGLAPLLNLWAKPQGR

SEQ ID NO: 948 - protein, 8 aa, Homo sapiens
IPSNPSHR

SEQ ID NO: 949 - protein, 15 aa, Homo sapiens
ANLINNIFELAGLGK

SEQ ID NO: 950 - protein, 11 aa, Homo sapiens
NEPEETPSIEK

SEQ ID NO: 951 - protein, 9 aa, Homo sapiens
VPSHAVVAR

SEQ ID NO: 952 - protein, 19 aa, Homo sapiens
GGLFADIASHPWQAAIFAK

SEQ ID NO: 953 - protein, 7 aa, Homo sapiens
SPQAFYR

SEQ ID NO: 954 - protein, 19 aa, Homo sapiens
SSNNPHSPIVEEFQVPYNK

SEQ ID NO: 955 - protein, 10 aa, Homo sapiens
LIEIANHVDK

SEQ ID NO: 956 - protein, 8 aa, Homo sapiens
GYQELLEK

SEQ ID NO: 957 - protein, 20 aa, Homo sapiens
SVVLIPLGAVDDGEHSQNEK

SEQ ID NO: 958 - protein, 18 aa, Homo sapiens
SETEIHQGFQHLHQLFAK

SEQ ID NO: 959 - protein, 8 aa, Homo sapiens
AEIEYLEK

SEQ ID NO: 960 - protein, 9 aa, Homo sapiens
VGVISFAQK

SEQ ID NO: 961 - protein, 17 aa, Homo sapiens
VFQYIDLHQDEFVQTLK

SEQ ID NO: 962 - protein, 8 aa, Homo sapiens
VLSSIEQK

SEQ ID NO: 963 - protein, 6 aa, Homo sapiens
TLPFSR

SEQ ID NO: 964 - protein, 16 aa, Homo sapiens
AEVIWTSSDHQVLSGK

SEQ ID NO: 965 - protein, 10 aa, Homo sapiens
YWGVASFLQK

SEQ ID NO: 966 - protein, 14 aa, Homo sapiens
SYTITGLQPGTDYK

SEQ ID NO: 967 - protein, 24 aa, Homo sapiens
ALNFGGIGVVVGHELTHAFDDQGR

SEQ ID NO: 968 - protein, 18 aa, Homo sapiens
SVPVTKPVPVTKPITVTK

SEQ ID NO: 969 - protein, 7 aa, Homo sapiens
IYLQPGR

SEQ ID NO: 970 - protein, 15 aa, Homo sapiens
EWVAIESDSVQPVPR

SEQ ID NO: 971 - protein, 25 aa, Homo sapiens
DLYHYITSYVVDGEIIIYGPAYSGR

SEQ ID NO: 972 - protein, 8 aa, Homo sapiens
ECEELEEK

SEQ ID NO: 973 - protein, 8 aa, Homo sapiens
STPSLTTK

SEQ ID NO: 974 - protein, 10 aa, Homo sapiens
ALLLGWVPTR

SEQ ID NO: 975 - protein, 14 aa, Homo sapiens
IALGGLLFPASNLR

SEQ ID NO: 976 - protein, 11 aa, Homo sapiens
GYVIIKPLVWV

SEQ ID NO: 977 - protein, 14 aa, Homo sapiens
NTGVISVVTTGLDR

SEQ ID NO: 978 - protein, 10 aa, Homo sapiens
SERPPIFEIR

SEQ ID NO: 979 - protein, 25 aa, Homo sapiens
TAHISGLPPSTDFIVYLSGLAPSIR

SEQ ID NO: 980 - protein, 9 aa, Homo sapiens
ATNATLDPR

SEQ ID NO: 981 - protein, 10 aa, Homo sapiens
QTLSWTVTPK

SEQ ID NO: 982 - protein, 9 aa, Homo sapiens
DIIKPDPPK

SEQ ID NO: 983 - protein, 6 aa, Homo sapiens
HVVQLR

SEQ ID NO: 984 - protein, 11 aa, Homo sapiens
NTVISVNPSTK

SEQ ID NO: 985 - protein, 7 aa, Homo sapiens
ILTPEVR

SEQ ID NO: 986 - protein, 7 aa, Homo sapiens
ELANTIK

SEQ ID NO: 987 - protein, 9 aa, Homo sapiens
LSIPQITTK

SEQ ID NO: 988 - protein, 17 aa, Homo sapiens
SVQNDSQAIAEVLNQLK

SEQ ID NO: 989 - protein, 14 aa, Homo sapiens
ALPGEQQPLHALTR

SEQ ID NO: 990 - protein, 18 aa, Homo sapiens
GTYLYNDCPGPGQDTDCR

SEQ ID NO: 991 - protein, 19 aa, Homo sapiens
NNQLVAGYLQGPNVNLEEK

SEQ ID NO: 992 - protein, 8 aa, Homo sapiens
FGSDDEGR

SEQ ID NO: 993 - protein, 13 aa, Homo sapiens
FATTFYQHLADSK

SEQ ID NO: 994 - protein, 10 aa, Homo sapiens
ETLALLSTHR

SEQ ID NO: 995 - protein, 6 aa, Homo sapiens
TYNVDK

SEQ ID NO: 996 - protein, 8 aa, Homo sapiens
LFIPQITR

SEQ ID NO: 997 - protein, 19 aa, Homo sapiens
NAVVQGLEQPHGLVVHPLR

SEQ ID NO: 998 - protein, 10 aa, Homo sapiens
AGFAGDDAPR

SEQ ID NO: 999 - protein, 9 aa, Homo sapiens
VIAVNEVGR

SEQ ID NO: 1000 - protein, 10 aa, Homo sapiens
SLSQQIENIR

SEQ ID NO: 1001 - protein, 7 aa, Homo sapiens
SVDEALR

SEQ ID NO: 1002 - protein, 12 aa, Homo sapiens
FVFGTTPEDILR

SEQ ID NO: 1003 - protein, 10 aa, Homo sapiens
TGYYFDGISR

SEQ ID NO: 1004 - protein, 9 aa, Homo sapiens
IGKPAPDFK

SEQ ID NO: 1005 - protein, 7 aa, Homo sapiens
FIVGFTR

SEQ ID NO: 1006 - protein, 14 aa, Homo sapiens
DSPVLIDFFEDTER

SEQ ID NO: 1007 - protein, 13 aa, Homo sapiens
VAPGVANPGTPLA

SEQ ID NO: 1008 - protein, 16 aa, Homo sapiens
NYFTSVAHPNLFIATK

SEQ ID NO: 1009 - protein, 9 aa, Homo sapiens
DTYVSSFPR

SEQ ID NO: 1010 - protein, 9 aa, Homo sapiens
HSHESQDLR

SEQ ID NO: 1011 - protein, 16 aa, Homo sapiens
VSFSSPLVAISGVALR

SEQ ID NO: 1012 - protein, 7 aa, Homo sapiens
WGAAPYR

SEQ ID NO: 1013 - protein, 14 aa, Homo sapiens
ALFLDALGPPAVTR

SEQ ID NO: 1014 - protein, 9 aa, Homo sapiens
AKPALEDLR

SEQ ID NO: 1015 - protein, 8 aa, Homo sapiens
VNFTEIQK

SEQ ID NO: 1016 - protein, 17 aa, Homo sapiens
GVTSVSQIFHSPDLAIR

SEQ ID NO: 1017 - protein, 10 aa, Homo sapiens
LLDSLPSDTR

SEQ ID NO: 1018 - protein, 10 aa, Homo sapiens
FQPTLLTLPR

SEQ ID NO: 1019 - protein, 8 aa, Homo sapiens
TLYSSSPR

SEQ ID NO: 1020 - protein, 15 aa, Homo sapiens
GDSGGAFAVQDPNDK

SEQ ID NO: 1021 - protein, 6 aa, Homo sapiens
LQVLGK

SEQ ID NO: 1022 - protein, 9 aa, Homo sapiens
LFIPQITPK

SEQ ID NO: 1023 - protein, 13 aa, Homo sapiens
IRPHTFTGLSGLR

SEQ ID NO: 1024 - protein, 11 aa, Homo sapiens
LSNENHGIAQR

SEQ ID NO: 1025 - protein, 9 aa, Homo sapiens
LHKPGVYTR

SEQ ID NO: 1026 - protein, 17 aa, Homo sapiens
TTIEKPVWLGFLGPIIK

SEQ ID NO: 1027 - protein, 10 aa, Homo sapiens
TQIDSPLSGK

SEQ ID NO: 1028 - protein, 11 aa, Homo sapiens
ATWSGAVLAGR

SEQ ID NO: 1029 - protein, 18 aa, Homo sapiens
VAPEEHPVLLTEAPLNPK

SEQ ID NO: 1030 - protein, 13 aa, Homo sapiens
CQCLQTLQGIHLK

SEQ ID NO: 1031 - protein, 10 aa, Homo sapiens
LLDFEFSSGR

SEQ ID NO: 1032 - protein, 14 aa, Homo sapiens
ILNTPNCALQIVAR

SEQ ID NO: 1033 - protein, 8 aa, Homo sapiens
GLFIIDGK

SEQ ID NO: 1034 - protein, 9 aa, Homo sapiens
EHSSLAFWK

SEQ ID NO: 1035 - protein, 8 aa, Homo sapiens
TFTLLDPK

SEQ ID NO: 1036 - protein, 13 aa, Homo sapiens
AHQLAIDTYQEFR

SEQ ID NO: 1037 - protein, 11 aa, Homo sapiens
AQETSGEEISK

SEQ ID NO: 1038 - protein, 10 aa, Homo sapiens
LSITGTYDLK

SEQ ID NO: 1039 - protein, 11 aa, Homo sapiens
EALVPLVADHK

SEQ ID NO: 1040 - protein, 12 aa, Homo sapiens
CRPINATLAVEK

SEQ ID NO: 1041 - protein, 12 aa, Homo sapiens
LTLLAPLNSVFK

SEQ ID NO: 1042 - protein, 16 aa, Homo sapiens
ADLFYDVEALDLESPK

SEQ ID NO: 1043 - protein, 10 aa, Homo sapiens
RIPLDLVPKT

SEQ ID NO: 1044 - protein, 20 aa, Homo sapiens
KENPAVIDFELAPIVDLVRN

SEQ ID NO: 1045 - protein, 20 aa, Homo sapiens
KYNPVVIDFEMQPIHEVLRH

SEQ ID NO: 1046 - protein, 13 aa, Homo sapiens
RGDSGGPLIVHKR

SEQ ID NO: 1047 - protein, 33 aa, Homo sapiens
RVLKDQVNTFDNIFIAPVGISTAMGMISLGLKG

SEQ ID NO: 1048 - protein, 17 aa, Homo sapiens
KPLLNDSRMLLSPDQKV

SEQ ID NO: 1049 - protein, 15 aa, Homo sapiens
KEDFTSLSLVLYSRK

SEQ ID NO: 1050 - protein, 14 aa, Homo sapiens
WNFAYWAAHQPWSR

SEQ ID NO: 1051 - protein, 11 aa, Homo sapiens
SEYGAALAWEK

SEQ ID NO: 1052 - protein, 13 aa, Homo sapiens
LWAYLTIQELLAK

SEQ ID NO: 1053 - protein, 8 aa, Homo sapiens
LLEVPEGR

SEQ ID NO: 1054 - protein, 10 aa, Homo sapiens
LTTVDIVTLR

SEQ ID NO: 1055 - protein, 6 aa, Homo sapiens
TLAFVR

SEQ ID NO: 1056 - protein, 9 aa, Homo sapiens
NSDQEIDFK

SEQ ID NO: 1057 - protein, 25 aa, Homo sapiens
YHFEALADTGISSEFYDNANDLLSK

SEQ ID NO: 1058 - protein, 20 aa, Homo sapiens
ILLLGTAVESAWGDEQSAFR

SEQ ID NO: 1059 - protein, 6 aa, Homo sapiens
YNQLLR

SEQ ID NO: 1060 - protein, 14 aa, Homo sapiens
VPGLYYFTYHASSR

SEQ ID NO: 1061 - protein, 8 aa, Homo sapiens
YGIEEHGK

SEQ ID NO: 1062 - protein, 13 aa, Homo sapiens
QVCADPSEEWVQK

SEQ ID NO: 1063 - protein, 11 aa, Homo sapiens
DPNGLPPEAQK

SEQ ID NO: 1064 - protein, 8 aa, Homo sapiens
ETLLQDFR

SEQ ID NO: 1065 - protein, 16 aa, Homo sapiens
IIEVEEEQEDPYLNDR

SEQ ID NO: 1066 - protein, 7 aa, Homo sapiens
ELCLDPK

SEQ ID NO: 1067 - protein, 11 aa, Homo sapiens
NQSPVLEPVGR

SEQ ID NO: 1068 - protein, 8 aa, Homo sapiens
FFQYDTWK

SEQ ID NO: 1069 - protein, 13 aa, Homo sapiens
SLQNASAIESILK